European Patent Application EP 4 431 527 A1, published September 18, 2024. Title: Fusion protein for localized activation of T-cells. Applicant: Medizinische Hochschule Hannover. The sequence listing filed with the application follows.

SEQUENCE LISTING (80 sequences)

SEQ ID NO: 1 - protein, 530 aa, synthetic construct
  SIGNAL 1..21: note = secretory leader
  CHAIN 24..129: note = anti-CD3 variable light chain
  CHAIN 130..144: note = linker
  CHAIN 145..263: note = anti-CD3 variable heavy chain
  CHAIN 264..273: note = linker
  CHAIN 279..284: note = 6x His Tag
  CHAIN 285..520: note = hinge
  CHAIN 521..530: note = HIV-Tat domain
MALLLCFVLLCGVVDFARSLSASDIQLTQSPAIMSASPGEKVTMTCRASSSVSYMNWYQQKSGTSPKRWIYDTSKVASGVPYRFSGSGSGTSYSLTISSMEAEDAATYYCQQWSSNPLTFGAGTKLELKGGGGSGGGGSGGGGSDIKLQQSGAELARPGASVKMSCKTSGYTFTRYTMHWVKQRPGQGLEWIGYINPSRGYTNYNQKFKDKATLTTDKSSSTAYMQLSSLTSEDSAVYYCARYYDDHYCLDYWGQGTTLTVSSEQKLISEEDLNMHTGHHHHHHPRGPTIKPCPPCKECHKCPAPNLEGGPSVFIFPPNIKDVLMISLTPKVTCVVVDVSEDDPDVRISWFVNNVEVHTAQTQTHREDYNSTIRVVSALPIQHQDWMSGKEFKCKVNNKDLPSPIERTISKIKGLVRAPQVYILPPPAEQLSRKDVSLTCLVVGFNPGDISVEWTSNGHTEENYKDTAPVLDSDGSYFIYSKLDIKTSKWEKTDSFSCNVRHEGLKNYYLKKTISRTPGKGRKKRRQRRR

SEQ ID NO: 2 - protein, 566 aa, synthetic construct
  SIGNAL 1..21: note = secretory leader
  CHAIN 24..129: note = anti-CD3 variable light chain
  CHAIN 130..144: note = Gly-Ser linker
  CHAIN 145..263: note = anti-CD3 variable heavy chain
  CHAIN 264..273: note = linker
  CHAIN 279..284: note = 6x His Tag
  CHAIN 285..520: note = hinge
  CHAIN 521..550: note = fibritin domain
  CHAIN 557..566: note = HIV-Tat domain
  CHAIN 551..556: note = spacer
MALLLCFVLLCGVVDFARSLSASDIQLTQSPAIMSASPGEKVTMTCRASSSVSYMNWYQQKSGTSPKRWIYDTSKVASGVPYRFSGSGSGTSYSLTISSMEAEDAATYYCQQWSSNPLTFGAGTKLELKGGGGSGGGGSGGGGSDIKLQQSGAELARPGASVKMSCKTSGYTFTRYTMHWVKQRPGQGLEWIGYINPSRGYTNYNQKFKDKATLTTDKSSSTAYMQLSSLTSEDSAVYYCARYYDDHYCLDYWGQGTTLTVSSEQKLISEEDLNMHTGHHHHHHPRGPTIKPCPPCKECHKCPAPNLEGGPSVFIFPPNIKDVLMISLTPKVTCVVVDVSEDDPDVRISWFVNNVEVHTAQTQTHREDYNSTIRVVSALPIQHQDWMSGKEFKCKVNNKDLPSPIERTISKIKGLVRAPQVYILPPPAEQLSRKDVSLTCLVVGFNPGDISVEWTSNGHTEENYKDTAPVLDSDGSYFIYSKLDIKTSKWEKTDSFSCNVRHEGLKNYYLKKTISRTPGKGYIPEAPRDGQAYVRKDGEWVLLSTFLSPAGGGGSGGRKKRRQRRR

SEQ ID NO: 3 - protein, 530 aa, synthetic construct
  SIGNAL 1..21: note = secretory leader
  CHAIN 24..142: note = anti-CD3 variable heavy chain
  CHAIN 143..157: note = Gly-Ser linker
  CHAIN 158..263: note = anti-CD3 variable light chain
  CHAIN 264..273: note = linker
  CHAIN 279..283: note = 6x His tag
  CHAIN 285..520: note = hinge
  CHAIN 521..530: note = HIV-Tat domain
MALLLCFVLLCGVVDFARSLSASDIKLQQSGAELARPGASVKMSCKTSGYTFTRYTMHWVKQRPGQGLEWIGYINPSRGYTNYNQKFKDKATLTTDKSSSTAYMQLSSLTSEDSAVYYCARYYDDHYCLDYWGQGTTLTVSSGGGGSGGGGSGGGGSDIQLTQSPAIMSASPGEKVTMTCRASSSVSYMNWYQQKSGTSPKRWIYDTSKVASGVPYRFSGSGSGTSYSLTISSMEAEDAATYYCQQWSSNPLTFGAGTKLELKEQKLISEEDLNMHTGHHHHHHPRGPTIKPCPPCKECHKCPAPNLEGGPSVFIFPPNIKDVLMISLTPKVTCVVVDVSEDDPDVRISWFVNNVEVHTAQTQTHREDYNSTIRVVSALPIQHQDWMSGKEFKCKVNNKDLPSPIERTISKIKGLVRAPQVYILPPPAEQLSRKDVSLTCLVVGFNPGDISVEWTSNGHTEENYKDTAPVLDSDGSYFIYSKLDIKTSKWEKTDSFSCNVRHEGLKNYYLKKTISRTPGKGRKKRRQRRR

SEQ ID NO: 4 - protein, 566 aa, synthetic construct
  SIGNAL 1..21: note = secretory leader
  CHAIN 24..142: note = anti-CD3 variable heavy chain
  CHAIN 143..157: note = Gly-Ser linker
  CHAIN 158..263: note = anti-CD3 variable light chain
  CHAIN 264..273: note = linker
  CHAIN 279..284: note = 6x His Tag
  CHAIN 285..520: note = hinge
  CHAIN 521..560: note = fibritin domain
  CHAIN 557..566: note = HIV-Tat domain
  CHAIN 551..556: note = spacer
MALLLCFVLLCGVVDFARSLSASDIKLQQSGAELARPGASVKMSCKTSGYTFTRYTMHWVKQRPGQGLEWIGYINPSRGYTNYNQKFKDKATLTTDKSSSTAYMQLSSLTSEDSAVYYCARYYDDHYCLDYWGQGTTLTVSSGGGGSGGGGSGGGGSDIQLTQSPAIMSASPGEKVTMTCRASSSVSYMNWYQQKSGTSPKRWIYDTSKVASGVPYRFSGSGSGTSYSLTISSMEAEDAATYYCQQWSSNPLTFGAGTKLELKEQKLISEEDLNMHTGHHHHHHPRGPTIKPCPPCKECHKCPAPNLEGGPSVFIFPPNIKDVLMISLTPKVTCVVVDVSEDDPDVRISWFVNNVEVHTAQTQTHREDYNSTIRVVSALPIQHQDWMSGKEFKCKVNNKDLPSPIERTISKIKGLVRAPQVYILPPPAEQLSRKDVSLTCLVVGFNPGDISVEWTSNGHTEENYKDTAPVLDSDGSYFIYSKLDIKTSKWEKTDSFSCNVRHEGLKNYYLKKTISRTPGKGYIPEAPRDGQAYVRKDGEWVLLSTFLSPAGGGGSGGRKKRRQRRR

SEQ ID NO: 5 - DNA, 1593 bp, synthetic construct
  source 1..1593: mol_type = other DNA
  CDS 1..69: protein_id = 14; translation = MALLLCFVLLCGVVDFARSLSAS
  CDS 70..387: note = anti-CD3 variable light chain; protein_id = 15; translation = DIQLTQSPAIMSASPGEKVTMTCRASSSVSYMNWYQQKSGTSPKRWIYDTSKVASGVPYRFSGSGSGTSYSLTISSMEAEDAATYYCQQWSSNPLTFGAGTKLELK
  CDS 388..432: note = GlySer linker; protein_id = 16; translation = GGGGSGGGGSGGGGS
  CDS 433..789: note = anti-CD3 variable heavy chain; protein_id = 17; translation = DIKLQQSGAELARPGASVKMSCKTSGYTFTRYTMHWVKQRPGQGLEWIGYINPSRGYTNYNQKFKDKATLTTDKSSSTAYMQLSSLTSEDSAVYYCARYYDDHYCLDYWGQGTTLTVSS
  CDS 790..852: note = mycHis tag; protein_id = 18; translation = EQKLISEEDLNMHTGHHHHHH
  CDS 853..1560: note = hinge; protein_id = 19; translation = PRGPTIKPCPPCKECHKCPAPNLEGGPSVFIFPPNIKDVLMISLTPKVTCVVVDVSEDDPDVRISWFVNNVEVHTAQTQTHREDYNSTIRVVSALPIQHQDWMSGKEFKCKVNNKDLPSPIERTISKIKGLVRAPQVYILPPPAEQLSRKDVSLTCLVVGFNPGDISVEWTSNGHTEENYKDTAPVLDSDGSYFIYSKLDIKTSKWEKTDSFSCNVRHEGLKNYYLKKTISRTPGK
  CDS 1561..1590: note = HIV-Tat domain; protein_id = 20; translation = GRKKRRQRRR
  CDS 1..1590: note = secretory leader peptide - human anti-CD3-scFv - Tag - hinge - HIV-Tat; protein_id = 61; translation = MALLLCFVLLCGVVDFARSLSASDIQLTQSPAIMSASPGEKVTMTCRASSSVSYMNWYQQKSGTSPKRWIYDTSKVASGVPYRFSGSGSGTSYSLTISSMEAEDAATYYCQQWSSNPLTFGAGTKLELKGGGGSGGGGSGGGGSDIKLQQSGAELARPGASVKMSCKTSGYTFTRYTMHWVKQRPGQGLEWIGYINPSRGYTNYNQKFKDKATLTTDKSSSTAYMQLSSLTSEDSAVYYCARYYDDHYCLDYWGQGTTLTVSSEQKLISEEDLNMHTGHHHHHHPRGPTIKPCPPCKECHKCPAPNLEGGPSVFIFPPNIKDVLMISLTPKVTCVVVDVSEDDPDVRISWFVNNVEVHTAQTQTHREDYNSTIRVVSALPIQHQDWMSGKEFKCKVNNKDLPSPIERTISKIKGLVRAPQVYILPPPAEQLSRKDVSLTCLVVGFNPGDISVEWTSNGHTEENYKDTAPVLDSDGSYFIYSKLDIKTSKWEKTDSFSCNVRHEGLKNYYLKKTISRTPGKGRKKRRQRRR
atggccctcctgctgtgcttcgtgctcctgtgcggagtggtggatttcgccagaagtttgagtgctagcgacattcagctgacccagtctccagcaatcatgtctgcatctccaggggagaaggtcaccatgacctgcagagccagttcaagtgtaagttacatgaactggtaccagcagaagtcaggcacctcccccaaaagatggatttatgacacatccaaagtggcttctggagtcccttatcgcttcagtggcagtgggtctgggacctcatactctctcacaatcagcagcatggaggctgaagatgctgccacttattactgccaacagtggagtagtaacccgctcacgttcggtgctgggaccaagctggagctgaaaggtggtggtggttctggcggcggcggctccggtggtggtggttctgatatcaaactgcagcagtcaggggctgaactggcaagacctggggcctcagtgaagatgtcctgcaagacttctggctacacctttactaggtacacgatgcactgggtaaaacagaggcctggacagggtctggaatggattggatacattaatcctagccgtggttatactaattacaatcagaagttcaaggacaaggccacattgactacagacaaatcctccagcacagcctacatgcaactgagcagcctgacatctgaggactctgcagtctattactgtgcaagatattatgatgatcattactgccttgactactggggccaaggcaccactctcacagtctcctcagaacagaaactcatctcagaagaggatctgaatatgcataccggacatcatcaccatcaccatcccagagggcccacaatcaagccctgtcctccatgcaaggagtgtcacaaatgcccagctcctaacctcgagggcggaccatccgtcttcatcttccctccaaatatcaaggatgtgctcatgatctccctgacacccaaggtcacctgtgtggtggtggatgtgagcgaggatgacccagacgtccggatcagctggtttgtgaacaacgtggaagtgcacacagctcagacacagacccatagagaggattacaacagtactatccgggtggtcagtgccctccccatccagcaccaggactggatgagtggcaaggagttcaaatgcaaggtcaacaacaaagacctcccatcacccatcgagagaaccatctcaaaaattaaagggctggtcagagctccacaggtgtacatcttgcctccaccagcagagcagttgtccaggaaagatgtcagtctcacttgcctggtcgtgggcttcaaccctggagacatcagtgtggagtggaccagcaatgggcatacagaggagaactacaaggacaccgcaccagtcctggactctgacggctcttacttcatctacagcaagctcgatatcaaaacaagcaagtgggagaaaacagattccttctcatgcaacgtgagacacgagggcctgaaaaattactacctgaagaagaccatctcccggactcctggcaaaggcaggaagaagcggagacagcgacgaagatag

SEQ ID NO: 6 - DNA, 1701 bp, synthetic construct
  source 1..1701: mol_type = other DNA
  CDS 1..69: note = secretory leader; protein_id = 21; translation = MALLLCFVLLCGVVDFARSLSAS
  CDS 70..387: note = anti-CD3 variable light chain; protein_id = 22; translation = DIQLTQSPAIMSASPGEKVTMTCRASSSVSYMNWYQQKSGTSPKRWIYDTSKVASGVPYRFSGSGSGTSYSLTISSMEAEDAATYYCQQWSSNPLTFGAGTKLELK
  CDS 388..432: note = linker; protein_id = 23; translation = GGGGSGGGGSGGGGS
  CDS 433..789: note = anti-CD3 variable heavy chain; protein_id = 24; translation = DIKLQQSGAELARPGASVKMSCKTSGYTFTRYTMHWVKQRPGQGLEWIGYINPSRGYTNYNQKFKDKATLTTDKSSSTAYMQLSSLTSEDSAVYYCARYYDDHYCLDYWGQGTTLTVSS
  CDS 790..852: note = MycHis-Tag; protein_id = 25; translation = EQKLISEEDLNMHTGHHHHHH
  CDS 853..1650: note = Hinge; protein_id = 26; translation = PRGPTIKPCPPCKECHKCPAPNLEGGPSVFIFPPNIKDVLMISLTPKVTCVVVDVSEDDPDVRISWFVNNVEVHTAQTQTHREDYNSTIRVVSALPIQHQDWMSGKEFKCKVNNKDLPSPIERTISKIKGLVRAPQVYILPPPAEQLSRKDVSLTCLVVGFNPGDISVEWTSNGHTEENYKDTAPVLDSDGSYFIYSKLDIKTSKWEKTDSFSCNVRHEGLKNYYLKKTISRTPGKGYIPEAPRDGQAYVRKDGEWVLLSTFLSPA
  CDS 1669..1698: note = HIV Tat; protein_id = 27; translation = GRKKRRQRRR
  CDS 1651..1668: note = hydrophilic spacer; protein_id = 28; translation = GGGGSG
  CDS 1..1698: note = secretory leader peptide - human anti-CD3-scFv - Tag - hinge - fibritin - spacer - HIV-Tat; protein_id = 62; translation = MALLLCFVLLCGVVDFARSLSASDIQLTQSPAIMSASPGEKVTMTCRASSSVSYMNWYQQKSGTSPKRWIYDTSKVASGVPYRFSGSGSGTSYSLTISSMEAEDAATYYCQQWSSNPLTFGAGTKLELKGGGGSGGGGSGGGGSDIKLQQSGAELARPGASVKMSCKTSGYTFTRYTMHWVKQRPGQGLEWIGYINPSRGYTNYNQKFKDKATLTTDKSSSTAYMQLSSLTSEDSAVYYCARYYDDHYCLDYWGQGTTLTVSSEQKLISEEDLNMHTGHHHHHHPRGPTIKPCPPCKECHKCPAPNLEGGPSVFIFPPNIKDVLMISLTPKVTCVVVDVSEDDPDVRISWFVNNVEVHTAQTQTHREDYNSTIRVVSALPIQHQDWMSGKEFKCKVNNKDLPSPIERTISKIKGLVRAPQVYILPPPAEQLSRKDVSLTCLVVGFNPGDISVEWTSNGHTEENYKDTAPVLDSDGSYFIYSKLDIKTSKWEKTDSFSCNVRHEGLKNYYLKKTISRTPGKGYIPEAPRDGQAYVRKDGEWVLLSTFLSPAGGGGSGGRKKRRQRRR
atggccctcctgctgtgcttcgtgctcctgtgcggagtggtggatttcgccagaagtttgagtgctagcgacattcagctgacccagtctccagcaatcatgtctgcatctccaggggagaaggtcaccatgacctgcagagccagttcaagtgtaagttacatgaactggtaccagcagaagtcaggcacctcccccaaaagatggatttatgacacatccaaagtggcttctggagtcccttatcgcttcagtggcagtgggtctgggacctcatactctctcacaatcagcagcatggaggctgaagatgctgccacttattactgccaacagtggagtagtaacccgctcacgttcggtgctgggaccaagctggagctgaaaggtggtggtggttctggcggcggcggctccggtggtggtggttctgatatcaaactgcagcagtcaggggctgaactggcaagacctggggcctcagtgaagatgtcctgcaagacttctggctacacctttactaggtacacgatgcactgggtaaaacagaggcctggacagggtctggaatggattggatacattaatcctagccgtggttatactaattacaatcagaagttcaaggacaaggccacattgactacagacaaatcctccagcacagcctacatgcaactgagcagcctgacatctgaggactctgcagtctattactgtgcaagatattatgatgatcattactgccttgactactggggccaaggcaccactctcacagtctcctcagaacagaaactcatctcagaagaggatctgaatatgcataccggacatcatcaccatcaccatcccagagggcccacaatcaagccctgtcctccatgcaaggagtgtcacaaatgcccagctcctaacctcgagggcggaccatccgtcttcatcttccctccaaatatcaaggatgtgctcatgatctccctgacacccaaggtcacctgtgtggtggtggatgtgagcgaggatgacccagacgtccggatcagctggtttgtgaacaacgtggaagtgcacacagctcagacacagacccatagagaggattacaacagtactatccgggtggtcagtgccctccccatccagcaccaggactggatgagtggcaaggagttcaaatgcaaggtcaacaacaaagacctcccatcacccatcgagagaaccatctcaaaaattaaagggctggtcagagctccacaggtgtacatcttgcctccaccagcagagcagttgtccaggaaagatgtcagtctcacttgcctggtcgtgggcttcaaccctggagacatcagtgtggagtggaccagcaatgggcatacagaggagaactacaaggacaccgcaccagtcctggactctgacggctcttacttcatctacagcaagctcgatatcaaaacaagcaagtgggagaaaacagattccttctcatgcaacgtgagacacgagggcctgaaaaattactacctgaagaagaccatctcccggactcctggcaaaggttatattcctgaagctccaagagatgggcaagcttacgttcgtaaagatggcgaatgggtattactttctacctttttatcaccagcaggaggaggagggtccggaggcaggaagaagcggagacagcgacgaagatag

SEQ ID NO: 7 - DNA, 1593 bp, synthetic construct
  source 1..1593: mol_type = other DNA
  CDS 1..69: note = secretory leader; protein_id = 29; translation = MALLLCFVLLCGVVDFARSLSAS
  CDS 70..423: note = anti-CD3 variable heavy chain; protein_id = 30; translation = DIKLQQSGAELARPGASVKMSCKTSGYTFTRYTMHWVKQRPGQGLEWIGYINPSRGYTNYNQKFKDKATLTTDKSSSTAYMQLSSLTSEDSAVYYCARYYDDHYCLDYWGQGTTLTVS
  CDS 424..471: note = linker; protein_id = 31; translation = SGGGGSGGGGSGGGGS
  CDS 472..789: note = anti-CD3 variable light chain; protein_id = 32; translation = DIQLTQSPAIMSASPGEKVTMTCRASSSVSYMNWYQQKSGTSPKRWIYDTSKVASGVPYRFSGSGSGTSYSLTISSMEAEDAATYYCQQWSSNPLTFGAGTKLELK
  CDS 790..852: note = MycHis-Tag; protein_id = 33; translation = EQKLISEEDLNMHTGHHHHHH
  CDS 853..1560: note = hinge; protein_id = 34; translation = PRGPTIKPCPPCKECHKCPAPNLEGGPSVFIFPPNIKDVLMISLTPKVTCVVVDVSEDDPDVRISWFVNNVEVHTAQTQTHREDYNSTIRVVSALPIQHQDWMSGKEFKCKVNNKDLPSPIERTISKIKGLVRAPQVYILPPPAEQLSRKDVSLTCLVVGFNPGDISVEWTSNGHTEENYKDTAPVLDSDGSYFIYSKLDIKTSKWEKTDSFSCNVRHEGLKNYYLKKTISRTPGK
  CDS 1561..1590: note = HIV-Tat; protein_id = 35; translation = GRKKRRQRRR
  CDS 1..1590: note = secretory leader peptide - human anti-CD3-scFv - Tag - hinge - HIV-Tat; protein_id = 63; translation = MALLLCFVLLCGVVDFARSLSASDIKLQQSGAELARPGASVKMSCKTSGYTFTRYTMHWVKQRPGQGLEWIGYINPSRGYTNYNQKFKDKATLTTDKSSSTAYMQLSSLTSEDSAVYYCARYYDDHYCLDYWGQGTTLTVSSGGGGSGGGGSGGGGSDIQLTQSPAIMSASPGEKVTMTCRASSSVSYMNWYQQKSGTSPKRWIYDTSKVASGVPYRFSGSGSGTSYSLTISSMEAEDAATYYCQQWSSNPLTFGAGTKLELKEQKLISEEDLNMHTGHHHHHHPRGPTIKPCPPCKECHKCPAPNLEGGPSVFIFPPNIKDVLMISLTPKVTCVVVDVSEDDPDVRISWFVNNVEVHTAQTQTHREDYNSTIRVVSALPIQHQDWMSGKEFKCKVNNKDLPSPIERTISKIKGLVRAPQVYILPPPAEQLSRKDVSLTCLVVGFNPGDISVEWTSNGHTEENYKDTAPVLDSDGSYFIYSKLDIKTSKWEKTDSFSCNVRHEGLKNYYLKKTISRTPGKGRKKRRQRRR
atggccctcctgctgtgcttcgtgctcctgtgcggagtggtggatttcgccagaagtttgagtgctagcgatatcaaactgcagcagtcaggggctgaactggcaagacctggggcctcagtgaagatgtcctgcaagacttctggctacacctttactaggtacacgatgcactgggtaaaacagaggcctggacagggtctggaatggattggatacattaatcctagccgtggttatactaattacaatcagaagttcaaggacaaggccacattgactacagacaaatcctccagcacagcctacatgcaactgagcagcctgacatctgaggactctgcagtctattactgtgcaagatattatgatgatcattactgccttgactactggggccaaggcaccactctcacagtctcctcaggaggaggagggtctggagggggcggctccggagggggtggttctgacattcagctgacccagtctccagcaatcatgtctgcatctccaggggagaaggtcaccatgacctgcagagccagttcaagtgtaagttacatgaactggtaccagcagaagtcaggcacctcccccaaaagatggatttatgacacatccaaagtggcttctggagtcccttatcgcttcagtggcagtgggtctgggacctcatactctctcacaatcagcagcatggaggctgaagatgctgccacttattactgccaacagtggagtagtaacccgctcacgttcggtgctgggaccaagctggagctgaaagaacagaaactcatctcagaagaggatctgaatatgcataccggacatcatcaccatcaccatcccagagggcccacaatcaagccctgtcctccatgcaaggagtgtcacaaatgcccagctcctaacctcgagggcggaccatccgtcttcatcttccctccaaatatcaaggatgtgctcatgatctccctgacacccaaggtcacctgtgtggtggtggatgtgagcgaggatgacccagacgtccggatcagctggtttgtgaacaacgtggaagtgcacacagctcagacacagacccatagagaggattacaacagtactatccgggtggtcagtgccctccccatccagcaccaggactggatgagtggcaaggagttcaaatgcaaggtcaacaacaaagacctcccatcacccatcgagagaaccatctcaaaaattaaagggctggtcagagctccacaggtgtacatcttgcctccaccagcagagcagttgtccaggaaagatgtcagtctcacttgcctggtcgtgggcttcaaccctggagacatcagtgtggagtggaccagcaatgggcatacagaggagaactacaaggacaccgcaccagtcctggactctgacggctcttacttcatctacagcaagctcgatatcaaaacaagcaagtgggagaaaacagattccttctcatgcaacgtgagacacgagggcctgaaaaattactacctgaagaagaccatctcccggactcctggcaaaggcaggaagaagcggagacagcgacgaagatag

SEQ ID NO: 8 - DNA, 1701 bp, synthetic construct
  source 1..1701: mol_type = other DNA
  CDS 1..69: note = secretory leader; protein_id = 36; translation = MALLLCFVLLCGVVDFARSLSAS
  CDS 70..426: note = anti-CD3 variable heavy chain; protein_id = 37; translation = DIKLQQSGAELARPGASVKMSCKTSGYTFTRYTMHWVKQRPGQGLEWIGYINPSRGYTNYNQKFKDKATLTTDKSSSTAYMQLSSLTSEDSAVYYCARYYDDHYCLDYWGQGTTLTVSS
  CDS 427..471: note = Gly-Ser linker; protein_id = 38; translation = GGGGSGGGGSGGGGS
  CDS 472..789: note = anti-CD3 variable light chain; protein_id = 39; translation = DIQLTQSPAIMSASPGEKVTMTCRASSSVSYMNWYQQKSGTSPKRWIYDTSKVASGVPYRFSGSGSGTSYSLTISSMEAEDAATYYCQQWSSNPLTFGAGTKLELK
  CDS 790..852: note = MycHis Tag; protein_id = 40; translation = EQKLISEEDLNMHTGHHHHHH
  CDS 853..1560: note = hinge; protein_id = 41; translation = PRGPTIKPCPPCKECHKCPAPNLEGGPSVFIFPPNIKDVLMISLTPKVTCVVVDVSEDDPDVRISWFVNNVEVHTAQTQTHREDYNSTIRVVSALPIQHQDWMSGKEFKCKVNNKDLPSPIERTISKIKGLVRAPQVYILPPPAEQLSRKDVSLTCLVVGFNPGDISVEWTSNGHTEENYKDTAPVLDSDGSYFIYSKLDIKTSKWEKTDSFSCNVRHEGLKNYYLKKTISRTPGK
  CDS 1561..1659: note = fibritin; protein_id = 42; translation = GYIPEAPRDGQAYVRKDGEWVLLSTFLSPAGGG
  CDS 1651..1668: note = hydrophilic spacer; protein_id = 43; translation = GGGGSG
  CDS 1669..1698: note = HIV-Tat; protein_id = 44; translation = GRKKRRQRRR
  CDS 1..1698: note = secretory leader peptide - human anti-CD3-scFv - Tag - hinge - fibritin - spacer - HIV-Tat; protein_id = 64; translation = MALLLCFVLLCGVVDFARSLSASDIKLQQSGAELARPGASVKMSCKTSGYTFTRYTMHWVKQRPGQGLEWIGYINPSRGYTNYNQKFKDKATLTTDKSSSTAYMQLSSLTSEDSAVYYCARYYDDHYCLDYWGQGTTLTVSSGGGGSGGGGSGGGGSDIQLTQSPAIMSASPGEKVTMTCRASSSVSYMNWYQQKSGTSPKRWIYDTSKVASGVPYRFSGSGSGTSYSLTISSMEAEDAATYYCQQWSSNPLTFGAGTKLELKEQKLISEEDLNMHTGHHHHHHPRGPTIKPCPPCKECHKCPAPNLEGGPSVFIFPPNIKDVLMISLTPKVTCVVVDVSEDDPDVRISWFVNNVEVHTAQTQTHREDYNSTIRVVSALPIQHQDWMSGKEFKCKVNNKDLPSPIERTISKIKGLVRAPQVYILPPPAEQLSRKDVSLTCLVVGFNPGDISVEWTSNGHTEENYKDTAPVLDSDGSYFIYSKLDIKTSKWEKTDSFSCNVRHEGLKNYYLKKTISRTPGKGYIPEAPRDGQAYVRKDGEWVLLSTFLSPAGGGGSGGRKKRRQRRR
atggccctcctgctgtgcttcgtgctcctgtgcggagtggtggatttcgccagaagtttgagtgctagcgatatcaaactgcagcagtcaggggctgaactggcaagacctggggcctcagtgaagatgtcctgcaagacttctggctacacctttactaggtacacgatgcactgggtaaaacagaggcctggacagggtctggaatggattggatacattaatcctagccgtggttatactaattacaatcagaagttcaaggacaaggccacattgactacagacaaatcctccagcacagcctacatgcaactgagcagcctgacatctgaggactctgcagtctattactgtgcaagatattatgatgatcattactgccttgactactggggccaaggcaccactctcacagtctcctcaggaggaggagggtctggagggggcggctccggagggggtggttctgacattcagctgacccagtctccagcaatcatgtctgcatctccaggggagaaggtcaccatgacctgcagagccagttcaagtgtaagttacatgaactggtaccagcagaagtcaggcacctcccccaaaagatggatttatgacacatccaaagtggcttctggagtcccttatcgcttcagtggcagtgggtctgggacctcatactctctcacaatcagcagcatggaggctgaagatgctgccacttattactgccaacagtggagtagtaacccgctcacgttcggtgctgggaccaagctggagctgaaagaacagaaactcatctcagaagaggatctgaatatgcataccggacatcatcaccatcaccatcccagagggcccacaatcaagccctgtcctccatgcaaggagtgtcacaaatgcccagctcctaacctcgagggcggaccatccgtcttcatcttccctccaaatatcaaggatgtgctcatgatctccctgacacccaaggtcacctgtgtggtggtggatgtgagcgaggatgacccagacgtccggatcagctggtttgtgaacaacgtggaagtgcacacagctcagacacagacccatagagaggattacaacagtactatccgggtggtcagtgccctccccatccagcaccaggactggatgagtggcaaggagttcaaatgcaaggtcaacaacaaagacctcccatcacccatcgagagaaccatctcaaaaattaaagggctggtcagagctccacaggtgtacatcttgcctccaccagcagagcagttgtccaggaaagatgtcagtctcacttgcctggtcgtgggcttcaaccctggagacatcagtgtggagtggaccagcaatgggcatacagaggagaactacaaggacaccgcaccagtcctggactctgacggctcttacttcatctacagcaagctcgatatcaaaacaagcaagtgggagaaaacagattccttctcatgcaacgtgagacacgagggcctgaaaaattactacctgaagaagaccatctcccggactcctggcaaaggttatattcctgaagctccaagagatgggcaagcttacgttcgtaaagatggcgaatgggtattactttctacctttttatcaccagcaggaggaggagggtccggaggcaggaagaagcggagacagcgacgaagatag

SEQ ID NO: 9 - protein, 526 aa, synthetic construct
  SIGNAL 1..21: note = secretory leader
  CHAIN 22..128: note = anti-CD3 variable light chain
  CA_BIND 129..143: note = Gly-Ser linker
  CHAIN 144..259: note = anti-CD3 variable heavy chain
  CHAIN 260..269: note = Myc Tag
  CHAIN 275..280: note = 6x His Tag
  CHAIN 281..516: note = hinge
  CHAIN 517..526: note = HIV-Tat domain
MALLLCFVLLCGVVDFARSLSDIQMTQSPSSLPASLGDRVTINCQASQDISNYLNWYQQKPGKAPKLLIYYTNKLADGVPSRFSGSGSGRDSSFTISSLESEDIGSYYCQQYYNYPWTFGPGTKLEIKGGGGSGGGGSGGGGSEVQLVESGGGLVQPGKSLKLSCEASGFTFSGYGMHWVRQAPGRGLESVAYITSSSINIKYADAVKGRFTVSRDNAKNLLFLQMNILKSEDTAMYYCARFDWDKNYWGQGTMVTVSSEQKLISEEDLNMHTGHHHHHHPRGPTIKPCPPCKECHKCPAPNLEGGPSVFIFPPNIKDVLMISLTPKVTCVVVDVSEDDPDVRISWFVNNVEVHTAQTQTHREDYNSTIRVVSALPIQHQDWMSGKEFKCKVNNKDLPSPIERTISKIKGLVRAPQVYILPPPAEQLSRKDVSLTCLVVGFNPGDISVEWTSNGHTEENYKDTAPVLDSDGSYFIYSKLDIKTSKWEKTDSFSCNVRHEGLKNYYLKKTISRTPGKGRKKRRQRRR

SEQ ID NO: 10 - protein, 562 aa, synthetic construct
  SIGNAL 1..21: note = secretory leader
  CHAIN 22..128: note = anti-CD3 variable light chain
  CHAIN 129..143: note = Gly-Ser linker
  CHAIN 144..259: note = anti-CD3 variable heavy chain
  CHAIN 260..269: note = Myc Tag
  CHAIN 275..280: note = 6x His Tag
  CHAIN 281..516: note = hinge
  CHAIN 517..552: note = fibritin domain
  CHAIN 553..562: note = HIV Tat domain
MALLLCFVLLCGVVDFARSLSDIQMTQSPSSLPASLGDRVTINCQASQDISNYLNWYQQKPGKAPKLLIYYTNKLADGVPSRFSGSGSGRDSSFTISSLESEDIGSYYCQQYYNYPWTFGPGTKLEIKGGGGSGGGGSGGGGSEVQLVESGGGLVQPGKSLKLSCEASGFTFSGYGMHWVRQAPGRGLESVAYITSSSINIKYADAVKGRFTVSRDNAKNLLFLQMNILKSEDTAMYYCARFDWDKNYWGQGTMVTVSSEQKLISEEDLNMHTGHHHHHHPRGPTIKPCPPCKECHKCPAPNLEGGPSVFIFPPNIKDVLMISLTPKVTCVVVDVSEDDPDVRISWFVNNVEVHTAQTQTHREDYNSTIRVVSALPIQHQDWMSGKEFKCKVNNKDLPSPIERTISKIKGLVRAPQVYILPPPAEQLSRKDVSLTCLVVGFNPGDISVEWTSNGHTEENYKDTAPVLDSDGSYFIYSKLDIKTSKWEKTDSFSCNVRHEGLKNYYLKKTISRTPGKGYIPEAPRDGQAYVRKDGEWVLLSTFLSPAGGGGSGGRKKRRQRRR

SEQ ID NO: 11 - DNA, 1581 bp, synthetic construct
  source 1..1581: mol_type = other DNA
  CDS 1..63: note = secretory leader; protein_id = 45; translation = MALLLCFVLLCGVVDFARSLS
  CDS 64..384: note = anti-CD3 variable light chain; protein_id = 46; translation = DIQMTQSPSSLPASLGDRVTINCQASQDISNYLNWYQQKPGKAPKLLIYYTNKLADGVPSRFSGSGSGRDSSFTISSLESEDIGSYYCQQYYNYPWTFGPGTKLEIK
  CDS 385..429: note = linker; protein_id = 47; translation = GGGGSGGGGSGGGGS
  CDS 430..777: note = anti-CD3 variable heavy chain; protein_id = 48; translation = EVQLVESGGGLVQPGKSLKLSCEASGFTFSGYGMHWVRQAPGRGLESVAYITSSSINIKYADAVKGRFTVSRDNAKNLLFLQMNILKSEDTAMYYCARFDWDKNYWGQGTMVTVSS
  CDS 778..840: note = MycHis Tag; protein_id = 49; translation = EQKLISEEDLNMHTGHHHHHH
  CDS 841..1548: note = hinge; protein_id = 50; translation = PRGPTIKPCPPCKECHKCPAPNLEGGPSVFIFPPNIKDVLMISLTPKVTCVVVDVSEDDPDVRISWFVNNVEVHTAQTQTHREDYNSTIRVVSALPIQHQDWMSGKEFKCKVNNKDLPSPIERTISKIKGLVRAPQVYILPPPAEQLSRKDVSLTCLVVGFNPGDISVEWTSNGHTEENYKDTAPVLDSDGSYFIYSKLDIKTSKWEKTDSFSCNVRHEGLKNYYLKKTISRTPGK
  CDS 1549..1578: note = HIV-Tat; protein_id = 51; translation = GRKKRRQRRR
  CDS 1..1578: note = secretory leader peptide - murine anti-CD3-scFv -Tag - hinge - HIV-Tat; protein_id = 65; translation = MALLLCFVLLCGVVDFARSLSDIQMTQSPSSLPASLGDRVTINCQASQDISNYLNWYQQKPGKAPKLLIYYTNKLADGVPSRFSGSGSGRDSSFTISSLESEDIGSYYCQQYYNYPWTFGPGTKLEIKGGGGSGGGGSGGGGSEVQLVESGGGLVQPGKSLKLSCEASGFTFSGYGMHWVRQAPGRGLESVAYITSSSINIKYADAVKGRFTVSRDNAKNLLFLQMNILKSEDTAMYYCARFDWDKNYWGQGTMVTVSSEQKLISEEDLNMHTGHHHHHHPRGPTIKPCPPCKECHKCPAPNLEGGPSVFIFPPNIKDVLMISLTPKVTCVVVDVSEDDPDVRISWFVNNVEVHTAQTQTHREDYNSTIRVVSALPIQHQDWMSGKEFKCKVNNKDLPSPIERTISKIKGLVRAPQVYILPPPAEQLSRKDVSLTCLVVGFNPGDISVEWTSNGHTEENYKDTAPVLDSDGSYFIYSKLDIKTSKWEKTDSFSCNVRHEGLKNYYLKKTISRTPGKGRKKRRQRRR
atggccctcctgctgtgcttcgtgctcctgtgcggagtggtggatttcgccagaagtttgagtgacatccagatgacccagtctccatcatcactgcctgcctccctgggagacagagtcactatcaattgtcaggccagtcaggacattagcaattatttgaactggtaccagcagaaaccagggaaagctcctaagctcctgatctattatacaaataaattggcagatggagtcccatcaaggttcagtggcagtggctctgggagagattcttctttcactatcagcagcctggaatccgaagatattggatcttattactgtcagcagtattataactatccctggaccttcggacctggcaccaagctggaaatcaaaggaggaggagggtccggagggggcggatctggagggggaggctctgaggtgcagctggtggagtctgggggaggcttggtgcagcctggaaagtccctgaaactctcctgtgaggcctctggattcaccttcagcggctatggcatgcactgggtccgccaggctccagggagggggctggagtccgtcgcatacattactagtagtagtattaatatcaaatatgctgacgctgtgaaaggccggttcaccgtctccagagacaatgccaagaacttgctgtttctgcagatgaacattctcaagtctgaggacacagccatgtactactgtgcaagattcgactgggacaaaaattactggggccagggaaccatggtcaccgtctcctcagaacagaaactcatctcagaagaggatctgaatatgcataccggacatcatcaccatcaccatcccagagggcccacaatcaagccctgtcctccatgcaaggagtgtcacaaatgcccagctcctaacctcgagggcggaccatccgtcttcatcttccctccaaatatcaaggatgtgctcatgatctccctgacacccaaggtcacctgtgtggtggtggatgtgagcgaggatgacccagacgtccggatcagctggtttgtgaacaacgtggaagtgcacacagctcagacacagacccatagagaggattacaacagtactatccgggtggtcagtgccctccccatccagcaccaggactggatgagtggcaaggagttcaaatgcaaggtcaacaacaaagacctcccatcacccatcgagagaaccatctcaaaaattaaagggctggtcagagctccacaggtgtacatcttgcctccaccagcagagcagttgtccaggaaagatgtcagtctcacttgcctggtcgtgggcttcaaccctggagacatcagtgtggagtggaccagcaatgggcatacagaggagaactacaaggacaccgcaccagtcctggactctgacggctcttacttcatctacagcaagctcgatatcaaaacaagcaagtgggagaaaacagattccttctcatgcaacgtgagacacgagggcctgaaaaattactacctgaagaagaccatctcccggactcctggcaaaggcaggaagaagcggagacagcgacgaagatag

SEQ ID NO: 12 - DNA, 1689 bp, synthetic construct
  source 1..1689: mol_type = other DNA
  CDS 1..63: note = secretory leader; protein_id = 52; translation = MALLLCFVLLCGVVDFARSLS
  CDS 64..384: note = anti-CD3 variable light chain; protein_id = 53; translation = DIQMTQSPSSLPASLGDRVTINCQASQDISNYLNWYQQKPGKAPKLLIYYTNKLADGVPSRFSGSGSGRDSSFTISSLESEDIGSYYCQQYYNYPWTFGPGTKLEIK
  CDS 385..429: note = linker; protein_id = 54; translation = GGGGSGGGGSGGGGS
  CDS 430..777: note = anti-CD3 variable heavy chain; protein_id = 55; translation = EVQLVESGGGLVQPGKSLKLSCEASGFTFSGYGMHWVRQAPGRGLESVAYITSSSINIKYADAVKGRFTVSRDNAKNLLFLQMNILKSEDTAMYYCARFDWDKNYWGQGTMVTVSS
  CDS 778..840: note = MycHis Tag; protein_id = 56; translation = EQKLISEEDLNMHTGHHHHHH
  CDS 841..1548: note = hinge; protein_id = 57; translation = PRGPTIKPCPPCKECHKCPAPNLEGGPSVFIFPPNIKDVLMISLTPKVTCVVVDVSEDDPDVRISWFVNNVEVHTAQTQTHREDYNSTIRVVSALPIQHQDWMSGKEFKCKVNNKDLPSPIERTISKIKGLVRAPQVYILPPPAEQLSRKDVSLTCLVVGFNPGDISVEWTSNGHTEENYKDTAPVLDSDGSYFIYSKLDIKTSKWEKTDSFSCNVRHEGLKNYYLKKTISRTPGK
  CDS 1549..1638: note = fibritin domain; protein_id = 58; translation = GYIPEAPRDGQAYVRKDGEWVLLSTFLSPA
  CDS 1639..1656: note = hydrophilic spacer; protein_id = 59; translation = GGGGSG
  CDS 1657..1686: note = HIV Tat domain; protein_id = 60; translation = GRKKRRQRRR
  CDS 1..1686: note = secretory leader peptide - human anti-CD3-scFv - Tag - hinge - fibritin - spacer - HIV-Tat; protein_id = 66; translation = MALLLCFVLLCGVVDFARSLSDIQMTQSPSSLPASLGDRVTINCQASQDISNYLNWYQQKPGKAPKLLIYYTNKLADGVPSRFSGSGSGRDSSFTISSLESEDIGSYYCQQYYNYPWTFGPGTKLEIKGGGGSGGGGSGGGGSEVQLVESGGGLVQPGKSLKLSCEASGFTFSGYGMHWVRQAPGRGLESVAYITSSSINIKYADAVKGRFTVSRDNAKNLLFLQMNILKSEDTAMYYCARFDWDKNYWGQGTMVTVSSEQKLISEEDLNMHTGHHHHHHPRGPTIKPCPPCKECHKCPAPNLEGGPSVFIFPPNIKDVLMISLTPKVTCVVVDVSEDDPDVRISWFVNNVEVHTAQTQTHREDYNSTIRVVSALPIQHQDWMSGKEFKCKVNNKDLPSPIERTISKIKGLVRAPQVYILPPPAEQLSRKDVSLTCLVVGFNPGDISVEWTSNGHTEENYKDTAPVLDSDGSYFIYSKLDIKTSKWEKTDSFSCNVRHEGLKNYYLKKTISRTPGKGYIPEAPRDGQAYVRKDGEWVLLSTFLSPAGGGGSGGRKKRRQRRR
atggccctcctgctgtgcttcgtgctcctgtgcggagtggtggatttcgccagaagtttgagtgacatccagatgacccagtctccatcatcactgcctgcctccctgggagacagagtcactatcaattgtcaggccagtcaggacattagcaattatttgaactggtaccagcagaaaccagggaaagctcctaagctcctgatctattatacaaataaattggcagatggagtcccatcaaggttcagtggcagtggctctgggagagattcttctttcactatcagcagcctggaatccgaagatattggatcttattactgtcagcagtattataactatccctggaccttcggacctggcaccaagctggaaatcaaaggaggaggagggtccggagggggcggatctggagggggaggctctgaggtgcagctggtggagtctgggggaggcttggtgcagcctggaaagtccctgaaactctcctgtgaggcctctggattcaccttcagcggctatggcatgcactgggtccgccaggctccagggagggggctggagtccgtcgcatacattactagtagtagtattaatatcaaatatgctgacgctgtgaaaggccggttcaccgtctccagagacaatgccaagaacttgctgtttctgcagatgaacattctcaagtctgaggacacagccatgtactactgtgcaagattcgactgggacaaaaattactggggccagggaaccatggtcaccgtctcctcagaacagaaactcatctcagaagaggatctgaatatgcataccggacatcatcaccatcaccatcccagagggcccacaatcaagccctgtcctccatgcaaggagtgtcacaaatgcccagctcctaacctcgagggcggaccatccgtcttcatcttccctccaaatatcaaggatgtgctcatgatctccctgacacccaaggtcacctgtgtggtggtggatgtgagcgaggatgacccagacgtccggatcagctggtttgtgaacaacgtggaagtgcacacagctcagacacagacccatagagaggattacaacagtactatccgggtggtcagtgccctccccatccagcaccaggactggatgagtggcaaggagttcaaatgcaaggtcaacaacaaagacctcccatcacccatcgagagaaccatctcaaaaattaaagggctggtcagagctccacaggtgtacatcttgcctccaccagcagagcagttgtccaggaaagatgtcagtctcacttgcctggtcgtgggcttcaaccctggagacatcagtgtggagtggaccagcaatgggcatacagaggagaactacaaggacaccgcaccagtcctggactctgacggctcttacttcatctacagcaagctcgatatcaaaacaagcaagtgggagaaaacagattccttctcatgcaacgtgagacacgagggcctgaaaaattactacctgaagaagaccatctcccggactcctggcaaaggttatattcctgaagctccaagagatgggcaagcttacgttcgtaaagatggcgaatgggtattactttctacctttttatcaccagcaggaggaggagggtccggaggcaggaagaagcggagacagcgacgaagatag

SEQ ID NO: 13 - DNA, 37135 bp, synthetic construct
  source 1..37135: mol_type = other DNA
  5'UTR 1..103: function = L-ITR
  3'UTR 37099..37135: function = R-ITR
  regulatory 380..625: regulatory_class = promoter
  gene 727..1646: gene = delta AA 4-25 variant of E1A gene
  misc_feature 837..857: note = RNAi target site
  misc_feature 886..909: note = RNAi target site
  misc_feature 1647..1764: note = heterologous target sites for RNAi inserted into the 3-UTR of E1A, equivalent to E1A-886-909, E1A-837-857, Prot IX-7467-7487
  regulatory 1813..1910: regulatory_class = promoter
  CDS 1911..2441: note = E1B-19k; protein_id = 67; translation = MEAWECLEDFSAVRNLLEQSSNSTSWFWRFLWGSSQAKLVCRIKEDYKWEFEELLKSCGELFDSLNLGHQALFQEKVIKTLDFSTPGRAAAAVAFLSFIKDKWSEETHLSGGYLLDFLAMHLWRAVVRHKNRLLLLSSVRPAIIPTEEQQQQQEEARRRRQEQSPWNPRAGLDPRE
  CDS 2216..3706: note = E1B-55k; protein_id = 68; translation = MERRNPSERGVPAGFSGHASVESGCETQESPATVVFRPPGDNTDGGAAAAAGGSQAAAAGAEPMEPESRPGPSGMNVVQVAELYPELRRILTITEDGQGLKGVKRERGACEATEEARNLAFSLMTRHRPECITFQQIKDNCANELDLLAQKYSIEQLTTYWLQPGDDFEEAIRVYAKVALRPDCKYKISKLVNIRNCCYISGNGAEVEIDTEDRVAFRCSMINMWPGVLGMDGVVIMNVRFTGPNFSGTVFLANTNLILHGVSFYGFNNTCVEAWTDVRVRGCAFYCCWKGVVCRPKSRASIKKCLFERCTLGILSEGNSRVRHNVASDCGCFMLVKSVAVIKHNMVCGNCEDRASQMLTCSDGNCHLLKTIHVASHSRKAWPVFEHNILTRCSLHLGNRRGVFLPYQCNLSHTKILLEPESMSKVNLNGVFDMTMKIWKVLRYDETRTRCRPCECGGKHIRNQPVMLDVTEELRPDHLVLACTRAEFGSSDEDTD
  regulatory 3737..4320: regulatory_class = ribosome_binding_site
  CDS 4339..5919: note = fusion protein; protein_id = 69; translation = MALLLCFVLLCGVVDFARSLSDIQMTQSPSSLPASLGDRVTINCQASQDISNYLNWYQQKPGKAPKLLIYYTNKLADGVPSRFSGSGSGRDSSFTISSLESEDIGSYYCQQYYNYPWTFGPGTKLEIKGGGGSGGGGSGGGGSEVQLVESGGGLVQPGKSLKLSCEASGFTFSGYGMHWVRQAPGRGLESVAYITSSSINIKYADAVKGRFTVSRDNAKNLLFLQMNILKSEDTAMYYCARFDWDKNYWGQGTMVTVSSEQKLISEEDLNMHTGHHHHHHPRGPTIKPCPPCKECHKCPAPNLEGGPSVFIFPPNIKDVLMISLTPKVTCVVVDVSEDDPDVRISWFVNNVEVHTAQTQTHREDYNSTIRVVSALPIQHQDWMSGKEFKCKVNNKDLPSPIERTISKIKGLVRAPQVYILPPPAEQLSRKDVSLTCLVVGFNPGDISVEWTSNGHTEENYKDTAPVLDSDGSYFIYSKLDIKTSKWEKTDSFSCNVRHEGLKNYYLKKTISRTPGKGRKKRRQRRR
  regulatory 5986..6344: note = prMinRGC; regulatory_class = promoter
  misc_feature 6439..6501: note = inhibitory shRNA for E1A
  misc_feature 6373..6435: note = inhibitory shRNA for E1A (1)
  misc_feature 6625..6681: note = inhibitory shRNA for Prot IX
  misc_feature 6748..6804: note = inhibitory shRNA for E4 orf6 (1)
  misc_feature 6936..6996: note = inhibitory shRNA for E4 orf6
  misc_feature 6996..7053: note = inhibitory shRNA for TP
  misc_feature 7120..7178: note = inhibitory shRNA for AdPol
  gene 7446..7868: note = protein IX, part of viral backbone
  gene 9034..17956: note = polymerase, Ad-Pol, part of viral backbone, reverse complementary
  gene 12420..17956: gene = terminal protein (TP), part of viral backbone, reverse complementary
  CDS 22677..25535: note = hexon, part of backbone; protein_id = 78; translation = MATPSMMPQWSYMHISGQDASEYLSPGLVQFARATETYFSLNNKFRNPTVAPTHDVTTDRSQRLTLRFIPVDREDTAYSYKARFTLAVGDNRVLDMASTYFDIRGVLDRGPTFKPYSGTAYNALAPKGAPNPCEWDEAATALEINLEEEDDDNEDEVDEQAEQQKTHVFGQAPYSGINITKEGIQIGVEGQTPKYADKTFQPEPQIGESQWYETEINHAAGRVLKKTTPMKPCYGSYAKPTNENGGQGILVKQQNGKLESQVEMQFFSTTEAAAGNGDNLTPKVVLYSEDVDIETPDTHISYMPTIKEGNSRELMGQQSMPNRPNYIAFRDNFIGLMYYNSTGNMGVLAGQASQLNAVVDLQDRNTELSYQLLLDSIGDRTRYFSMWNQAVDSYDPDVRIIENHGTEDELPNYCFPLGGVINTETLTKVKPKTGQENGWEKDATEFSDKNEIRVGNNFAMEINLNANLWRNFLYSNIALYLPDKLKYSPSNVKISDNPNTYDYMNKRVVAPGLVDCYINLGARWSLDYMDNVNPFNHHRNAGLRYRSMLLGNGRYVPFHIQVPQKFFAIKNLLLLPGSYTYEWNFRKDVNMVLQSSLGNDLRVDGASIKFDSICLYATFFPMAHNTASTLEAMLRNDTNDQSFNDYLSAANMLYPIPANATNVPISIPSRNWAAFRGWAFTRLKTKETPSLGSGYDPYYTYSGSIPYLDGTFYLNHTFKKVAITFDSSVSWPGNDRLLTPNEFEIKRSVDGEGYNVAQCNMTKDWFLVQMLANYNIGYQGFYIPESYKDRMYSFFRNFQPMSRQVVDDTKYKDYQQVGILHQHNNSGFVGYLAPTMREGQAYPANFPYPLIGKTAVDSITQKKFLCDRTLWRIPFSSNFMSMGALTDLGQNLLYANSAHALDMTFEVDPMDEPTLLYVLFEVFDVVRVHQPHRGVIETVYLRTPFSAGNATT
  gene 26280..27869: gene = reverse complementary sequence of DNA-binding protein (dbd), part of viral backbone
  misc_feature 31703: note = delta E3, equivalent to deletion of nt 28137..30818 of wildtype virus
  CDS 32222..33967: note = fiber, part of viral backbone; protein_id = 70; translation = MKRARPSEDTFNPVYPYDTETGPPTVPFLTPPFVSPNGFQESPPGVLSLRLSEPLVTSNGMLALKMGNGLSLDEAGNLTSQNVTTVSPPLKKTKSNINLEISAPLTVTSEALTVAAAAPLMVAGNTLTMQSQAPLTVHDSKLSIATQGPLTVSEGKLALQTSGPLTTTDSSTLTITASPPLTTATGSLGIDLKEPIYTQNGKLGLKYGAPLHVTDDLNTLTVATGPGVTINNTSLQTKVTGALGFDSQGNMQLNVAGGLRIDSQNRRLILDVSYPFDAQNQLNLRLGQGPLFINSAHNLDINYNKGLYLFTASNNSKKLEVNLSTAKGLMFDATAIAINAGDGLEFGSPNAPNTNPLKTKIGHGLEFDSNKAMVPKLGTGLSFDSTGAITVGNKNNDKLTLWTTPAPSPNCRLNAEKDAKLTLVLTKCGSQILATVSVLAVKGSLAPISGTVQSAHLIIRFDENGVLLNNSFLDPEYWNFRNGDLTEGTAYTNAVGFMPNLSAYPKSHGKTAKSNIVSQVYLNGDKTKPVTLTITLNGTQETGDTTPSAYSMSFSWDWSGHNYINEIFATSSYTFSYIAQE
  gene 34094..35257: gene = reverse complementary sequence of E4 orf6/7
  gene 35178..35492: gene = reverse complementary sequence of hybrid E4 orf4, Ad5/Ad11
  regulatory 35861..35863: regulatory_class = terminator
  misc_feature 35861..35884: note = inactivated E4 orf3 locus, reverse complementary
  gene 35881..36291: note = E4 orf2, reverse complementary
  gene 36321..36707: note = E4 orf1 reverse complementary
  misc_feature 37099..37135: note = LTR, r-ITR
  gene 27896..30319: gene = 100k, part of viral backbone
  misc_feature 6501..6558: note = inhibitory shRNA for E1A (2)
  misc_feature 6870..6930: note = inhibitory shRNA for E4 orf6 (2)
  CDS 17992..19707: note = Prot III: penton, part of backbone; protein_id = 77; translation = MRRAAMYEEGPPPSYESVVSAAPVAAALGSPFDAPLDPPFVPPRYLRPTGGRNSIRYSELAPLFDTTRVYLVDNKSTDVASLNYQNDHSNFLTTVIQNNDYSPGEASTQTINLDDRSHWGGDLKTILHTNMPNVNEFMFTNKFKARVMVSRLPTKDNQVELKYEWVEFTLPEGNYSETMTIDLMNNAIVEHYLKVGRQNGVLESDIGVKFDTRNFRLGFDPVTGLVMPGVYTNEAFHPDIILLPGCGVDFTHSRLSNLLGIRKRQPFQEGFRITYDDLEGGNIPALLDVDAYQASLKDDTEQGGGGAGGSNSSGSGAEENSNAAAAAMQPVEDMNDHAIRGDTFATRAEEKRAEAEAAAEAAAPAAQPEVEKPQKKPVIKPLTEDSKKRSYNLISNDSTFTQYRSWYLAYNYGDPQTGIRSWTLLCTPDVTCGSEQVYWSLPDMMQDPVTFRSTRQISNFPVVGAELLPVHSKSFYNDQAVYSQLIRQFTSLTHVFNRFPENQILARPPAPTITTVSENVPALTDHGTLPLRNSIGGVQRVTITDARRRTCPYVYKALGIVSPRVLSSRTF
catcatcaataatataccttattttggattgaagccaatatgataatgagggggtggagtttgtgacgtggcgcggggcgtgggaacggggcgggtgacgtagtagtgtggcggaagtgtgatgttgcaagtgtggcggaacacatgtaagcgacggatgtggcaaaagtgacgtttttggtgtgcgccggtgtacacaggaagtgacaattttcgcgcggttttaggcggatgttgtagtaaatttgggcgtaaccgagtaagatttggccattttcgcgggaaaactgaataagaggaagtgaaatctgaataattttgtgttactcatagcgcgtaatctctagcatcgtaactataacggtcctaaggtagcgaaagctagtaccatggtgatgcggttttggcagtacatcaatggcggtggatagcggtccgactcacggggatttccaagtctccaccccattgacgtcaatgggagtttgttttggcaccaaaatcaacgggactttccaaaatgtcgtaacaactccgccccacggacgcaaatgggccgtaggcgtgtacggtgggcggtctatataagcccggctggtttagtgaaccgtcagatcctcgagggcgtgtagtgtatttatacccggtgagttcctcaagaggccactcttgagtgccagcgagtagagttttctcctccgagccgctccgacaccgggactgaaaatgagacatgaggtactggctgataatcttccacctcctagccattttgaaccacctacccttcacgaactgtatgatttagacgtgacggcccccgaagatcccaacgaggaggcggtttcgcagatttttcccgactctgtaatgttggcggtgcaggaagggattgacttactcacttttccgccggcgcccggttctccggagccgcctcacctttcccggcagcccgagcagccggagcagagagccttgggtccggtttctatgccaaaccttgtaccggaggtgatcgatcttacctgccacgaggctggctttccacccagtgacgacgaggatgaagagggtgaggagtttgtgttagattatgtggagcaccccgggcacggttgcaggtcttgtcattatcaccggaggaatacgggggacccagatattatgtgttcgctttgctatatgaggacctgtggcatgtttgtctacagtaagtgaaaattatgggcagtgggtgatagagtggtgggtttggtgtggtaattttttttttaatttttacagttttgtggtttaaagaattttgtattgtgatttttttaaaaggtcctgtgtctgaacctgagcctgagcccgagccagaaccggagcctgcaagacctacccgccgtcctaaaatggcgcctgctatcctgagacgcccgacatcacctgtgtctagagaatgcaatagtagtacggatagctgtgactccggtccttctaacacacctcctgagatacacccggtggtcccgctgtgccccattaaaccagttgccgtgagagttggtgggcgtcgccaggctgtggaatgtatcgaggacttgcttaacgagcctgggcaacctttggacttgagctgtaaacgccccaggccataaggtgtaaacctgtgattgcgtgtgtggttaacacacaggaggcggtttcgcagatttttacacacagaagggattgacttactcacttttacacacaggaagcattgtgagctcatatgagacccaacgcctttgtttgctgaatgagttgatgtaagtttaataaagggtgagataatgtttaacttgcatggcgtgttaaatggggcggggcttaaagggtatataatgcgccgtgggctaatcttggttacatctgacctcatggaggcttgggagtgtttggaagatttttctgctgtgcgtaacttgctggaacagagctctaacagtacctcttggttttggaggtttctgtggggctcatcccaggcaaagttagtctgcagaattaaggaggattacaagtgggaatttgaagagcttttgaaatcctgtggtgagctgtttgattctttgaatctgggtcaccaggcgcttttccaagagaaggtcatcaagactttggatttttccacaccggggcgcgctgcggctgctgttgcttttttgagttttataaaggataaatggagcgaagaaacccatctgagcggggggtacctgctggattttctggccatgcatctgtggagagcggttgtgagacacaagaatcgcctgctactgttgtcttccgtccgcccggcgataataccgacggaggagcagcagcagcagcaggaggaagccaggcggcggcggcaggagcagagcccatggaacccgagagccggcctggaccctcgggaatgaatgttgtacaggtggctgaactgtatccagaactgagacgcattttgacaattacagaggatgggcaggggctaaagggggtaaagagggagcggggggcttgtgaggctacagaggaggctaggaatctagcttttagcttaatgaccagacaccgtcctgagtgtattacttttcaacagatcaaggataattgcgctaatgagcttgatctgctggcgcagaagtattccatagagcagctgaccacttactggctgcagccaggggatgattttgaggaggctattagggtatatgcaaaggtggcacttaggccagattgcaagtacaagatcagcaaacttgtaaatatcaggaattgttgctacatttctgggaacggggccgaggtggagatagatacggaggatagggtggcctttagatgtagcatgataaatatgtggccgggggtgcttggcatggacggggtggttattatgaatgtaaggtttactggccccaattttagcggtacggttttcctggccaataccaaccttatcctacacggtgtaagcttctatgggtttaacaatacctgtgtggaagcctggaccgatgtaagggttcggggctgtgccttttactgctgctggaagggggtggtgtgtcgccccaaaagcagggcttcaattaagaaatgcctctttgaaaggtgtaccttgggtatcctgtctgagggtaactccagggtgcgccacaatgtggcctccgactgtggttgcttcatgctagtgaaaagcgtggctgtgattaagcataacatggtatgtggcaactgcgaggacagggcctctcagatgctgacctgctcggacggcaactgtcacctgctgaagaccattcacgtagccagccactctcgcaaggcctggccagtgtttgagcataacatactgacccgctgttccttgcatttgggtaacaggaggggggtgttcctaccttaccaatgcaatttgagtcacactaagatattgcttgagcccgagagcatgtccaaggtgaacctgaacggggtgtttgacatgaccatgaagatctggaaggtgctgaggtacgatgagacccgcaccaggtgcagaccctgcgagtgtggcggtaaacatattaggaaccagcctgtgatgctggatgtgaccgaggagctgaggcccgatcacttggtgctggcctgcacccgcgctgagtttggctctagcgatgaagatacagattgaggtactgaaatgtgtgggcgtggcgaattccgcccctctccctcccccccccctaacgttactggccgaagccgcttggaataaggccggtgtgcgtttgtctatatgttattttccaccatattgccgtcttttggcaatgtgagggcccggaaacctggccctgtcttcttgacgagcattcctaggggtctttcccctctcgccaaaggaatgcaaggtctgttgaatgtcgtgaaggaagcagttcctctggaagcttcttgaagacaaacaacgtctgtagcgaccctttgcaggcagcggaaccccccacctggcgacaggtgcctctgcggccaaaagccacgtgtataagatacacctgcaaaggcggcacaaccccagtgccacgttgtgagttggatagttgtggaaagagtcaaatggctctcctcaagcgtattcaacaaggggctgaaggatgcccagaaggtaccccattgtatgggatctgatctggggcctcggtgcacatgctttacatgtgtttagtcgaggttaaaaaaacgtctaggccccccgaaccacggggacgtggttttcctttgaaaaacacgatgataagcttgatcacgcgtttcgaacgatttatggccctcctgctgtgcttcgtgctcctgtgcggagtggtggatttcgccagaagtttgagtgacatccagatgacccagtctccatcatcactgcctgcctccctgggagacagagtcactatcaattgtcaggccagtcaggacattagcaattatttgaactggtaccagcagaaaccagggaaagctcctaagctcctgatctattatacaaataaattggcagatggagtcccatcaaggttcagtggcagtggctctgggagagattcttctttcactatcagcagcctggaatccgaagatattggatcttattactgtcagcagtattataactatccctggaccttcggacctggcaccaagctggaaatcaaaggaggaggagggtccggagggggcggatctggagggggaggctctgaggtgcagctggtggagtctgggggaggcttggtgcagcctggaaagtccctgaaactctcctgtgaggcctctggattcaccttcagcggctatggcatgcactgggtccgccaggctccagggagggggctggagtccgtcgcatacattactagtagtagtattaatatcaaatatgctgacgctgtgaaaggccggttcaccgtctccagagacaatgccaagaacttgctgtttctgcagatgaacattctcaagtctgaggacacagccatgtactactgtgcaagattcgactgggacaaaaattactggggccagggaaccatggtcaccgtctcctcagaacagaaactcatctcagaagaggatctgaatatgcataccggacatcatcaccatcaccatcccagagggcccacaatcaagccctgtcctccatgcaaggagtgtcacaaatgcccagctcctaacctcgagggcggaccatccgtcttcatcttccctccaaatatcaaggatgtgctcatgatctccctgacacccaaggtcacctgtgtggtggtggatgtgagcgaggatgacccagacgtccggatcagctggtttgtgaacaacgtggaagtgcacacagctcagacacagacccatagagaggattacaacagtactatccgggtggtcagtgccctccccatccagcaccaggactggatgagtggcaaggagttcaaatgcaaggtcaacaacaaagacctcccatcacccatcgagagaaccatctcaaaaattaaagggctggtcagagctccacaggtgtacatcttgcctccaccagcagagcagttgtccaggaaagatgtcagtctcacttgcctggtcgtgggcttcaaccctggagacatcagtgtggagtggaccagcaatgggcatacagaggagaactacaaggacaccgcaccagtcctggactctgacggctcttacttcatctacagcaagctcgatatcaaaacaagcaagtgggagaaaacagattccttctcatgcaacgtgagacacgagggcctgaaaaattactacctgaagaagaccatctcccggactcctggcaaaggcaggaagaagcggagacagcgacgaagatagaaataaaggtaccttattttcattagatttgtgtgttggttttttgtgtggcggcctcgagatgggagagcttgatgccaggcaagtccaggcaggccaggcaagtccaggcaggccaggcaagtccaggcaggccaggcaagtccaggcaggccaggcaagtccaggcaggccaggcaagtccaggcaggccaggcaagtccaggcaggccaggcaagtccaggcaggccaggcaagtccaggcaggccaggcaagtccaggcagggccaggcaagtccaggcaggccaggcaagtccaggcaggccaggcaagtccaggcaggatcgaattcgagctcgtacggtgggagggctatataagcagacctcgtttagtgaaccgtcagatcgcctggagacgaagcttgctagcggatcctcgagaaggtatattgctgttgacagtgagcgagaagggattgacttactcacttttgtgaagccacagatgaaaagtgagtaagtcaatcccttcgtgcctactgcctcggaattcactagcggatcctcgagaaggtatattgctgttgacagtgagcgaggaggcggtttcgcagattttgtgaagccacagatgaaaatctgcgaaaccgcctccgtgcctactgcctcggaattcactagcggatcctcgagaaggtatattgctgttgacagtgagcgaggaagcattgtgagctcatatgtgaagccacagatgatatgagctcacaatgcttccgtgcctactgcctcggaattcactagcggatcctcgagaaggtatattgctgttgacagtgagcgagacaggaaaccgtgtggaatagtgaagccacagatgtattccacacggtttcctgtcgtgcctactgcctcggaattcactagcggatcctcgaaaggtatattgctgttgacagtgagcgaccatgtttaatcagaggtttatagtgaagccacagatgtataaacctctgattaaacatgggtgcctactgcctcggaattcactagcggatcctcgagaaggtatattgctgttgacagtgagcgacggagtacctacacaacaattgtgaagccacagatgaattgttgtgtaggtactccggtgcctactgcctcggaattcactagcggatcctcgagaaggtatattgctgttgacagtgagcgagcgaatacgtgcagctaaacatgtgaagccacagatgatgtttagctgcacgtattcgcgtgcctactgcctcggaattcactagctagtcatatgctgcagtgtagatctaaataaagcaatagcatcacaaataaagcatttcattcactgcattctagttgtggtttgtacgcgtgatatcaattcatctatgtcgggtgcggagaaagaggtaatgaaatggcatcgactcgaagatctgggcgtggttaagggtgggaaagaatatataaggtgggggtcttatgtagttttgtatctgttttgcagcagccgccgccgccatgagcaccaactcgtttgatggaagcattgtgagctcatatttgacaacgcgcatgcccccatgggccggggtgcgtcagaatgtgatgggctccagcattgatggtcgccccgtcctgcccgcaaactctactaccttgacctacgagaccgtgtctggaacgccgttggagactgcagcctccgccgccgcttcagccgctgcagccaccgcccgcgggattgtgactgactttgctttcctgagcccgcttgcaagcagtgcagcttcccgttcatccgcccgcgatgacaagttgacggctcttttggcacaattggattctttgacccgggaacttaatgtcgtttctcagcagctgttggatctgcgccagcaggtttctgccctgaaggcttcctcccctcccaatgcggtttaaaacataaataaaaaaccagactctgtttggatttggatcaagcaagtgtcttgctgtctttatttaggggttttgcgcgcgcggtaggcccgggaccagcggtctcggtcgttgagggtcctgtgtattttttccaggacgtggtaaaggtgactctggatgttcagatacatgggcataagcccgtctctggggtggaggtagcaccactgcagagcttcatgctgcggggtggtgttgtagatgatccagtcgtagcaggagcgctgggcgtggtgcctaaaaatgtctttcagtagcaagctgattgccaggggcaggcccttggtgtaagtgtttacaaagcggttaagctgggatgggtgcatacgtggggatatgagatgcatcttggactgtatttttaggttggctatgttcccagccatatccctccggggattcatgttgtgcagaaccaccagcacagtgtatccggtgcacttgggaaatttgtcatgtagcttagaaggaaatgcgtggaagaacttggagacgcccttgtgacctccaagattttccatgcattcgtccataatgatggcaatgggcccacgggcggcggcctgggcgaagatatttctgggatcactaacgtcatagttgtgttccaggatgagatcgtcataggccatttttacaaagcgcgggcggagggtgccagactgcggtataatggttccatccggcccaggggcgtagttaccctcacagatttgcatttcccacgctttgagttcagatggggggatcatgtctacctgcggggcgatgaagaaaacggtttccggggtaggggagatcagctgggaagaaagcaggttcctgagcagctgcgacttaccgcagccggtgggcccgtaaatcacacctattaccggctgcaactggtagttaagagagctgcagctgccgtcatccctgagcaggggggccacttcgttaagcatgtccctgactcgcatgttttccctgaccaaatccgccagaaggcgctcgccgcccagcgatagcagttcttgcaaggaagcaaagtttttcaacggtttgagaccgtccgccgtaggcatgcttttgagcgtttgaccaagcagttccaggcggtcccacagctcggtcacctgctctacggcatctcgatccagcatatctcctcgtttcgcgggttggggcggctttcgctgtacggcagtagtcggtgctcgtccagacgggccagggtcatgtctttccacgggcgcagggtcctcgtcagcgtagtctgggtcacggtgaaggggtgcgctccgggctgcgcgctggccagggtgcgcttgaggctggtcctgctggtgctgaagcgctgccggtcttcgccctgcgcgtcggccaggtagcatttgaccatggtgtcatagtccagcccctccgcggcgtggcccttggcgcgcagcttgcccttggaggaggcgccgcacgaggggcagtgcagacttttgagggcgtagagcttgggcgcgagaaataccgattccggggagtaggcatccgcgccgcaggccccgcagacggtctcgcattccacgagccaggtgagctctggccgttcggggtcaaaaaccaggtttcccccatgctttttgatgcgtttcttacctctggtttccatgagccggtgtccacgctcggtgacgaaaaggctgtccgtgtccccgtatacagacttgagaggcctgtcctcgagcggtgttccgcggtcctcctcgtatagaaactcggaccactctgagacaaaggctcgcgtccaggccagcacgaaggaggctaagtgggaggggtagcggtcgttgtccactagggggtccactcgctccagggtgtgaagacacatgtcgccctcttcggcatcaaggaaggtgattggtttgtaggtgtaggccacgtgaccgggtgttcctgaaggggggctataaaagggggtgggggcgcgttcgtcctcactctcttccgcatcgctgtctgcgagggccagctgttggggtgagtactccctctgaaaagcgggcatgacttctgcgctaagattgtcagtttccaaaaacgaggaggatttgatattcacctggcccgcggtgatgcctttgagggtggccgcatccatctggtcagaaaagacaatctttttgttgtcaagcttggtggcaaacgacccgtagagggcgttggacagcaacttggcgatggagcgcagggtttggtttttgtcgcgatcggcgcgctccttggccgcgatgtttagctgcacgtattcgcgcgcaacgcaccgccattcgggaaagacggtggtgcgctcgtcgggcaccaggtgcacgcgccaaccgcggttgtgcagggtgacaaggtcaacgctggtggctacctctccgcgtaggcgctcgttggtccagcagaggcggccgcccttgcgcgagcagaatggcggtagggggtctagctgcgtctcgtccggggggtctgcgtccacggtaaagaccccgggcagcaggcgcgcgtcgaagtagtctatcttgcatccttgcaagtctagcgcctgctgccatgcgcgggcggcaagcgcgcgctcgtatgggttgagtgggggaccccatggcatggggtgggtgagcgcggaggcgtacatgccgcaaatgtcgtaaacgtagaggggctctctgagtattccaagatatgtagggtagcatcttccaccgcggatgctggcgcgcacgtaatcgtatagttcgtgcgagggagcgaggaggtcgggaccgaggttgctacgggcgggctgctctgctcggaagactatctgcctgaagatggcatgtgagttggatgatatggttggacgctggaagacgttgaagctggcgtctgtgagacctaccgcgtcacgcacgaaggaggcgtaggagtcgcgcagcttgttgaccagctcggcggtgacctgcacgtctagggcgcagtagtccagggtttccttgatgatgtcatacttatcctgtcccttttttttccacagctcgcggttgaggacaaactcttcgcggtctttccagtactcttggatcggaaacccgtcggcctccgaacggtaagagcctagcatgtagaactggttgacggcctggtaggcgcagcatcccttttctacgggtagcgcgtatgcctgcgcggccttccggagcgaggtgtgggtgagcgcaaaggtgtccctgaccatgactttgaggtactggtatttgaagtcagtgtcgtcgcatccgccctgctcccagagcaaaaagtccgtgcgctttttggaacgcggatttggcagggcgaaggtgacatcgttgaagagtatctttcccgcgcgaggcataaagttgcgtgtgatgcggaagggtcccggcacctcggaacggttgttaattacctgggcggcgagcacgatctcgtcaaagccgttgatgttgtggcccacaatgtaaagttccaagaagcgcgggatgcccttgatggaaggcaattttttaagttcctcgtaggtgagctcttcaggggagctgagcccgtgctctgaaagggcccagtctgcaagatgagggttggaagcgacgaatgagctccacaggtcacgggccattagcatttgcaggtggtcgcgaaaggtcctaaactggcgacctatggccattttttctggggtgatgcagtagaaggtaagcgggtcttgttcccagcggtcccatccaaggttcgcggctaggtctcgcgcggcagtcactagaggctcatctccgccgaacttcatgaccagcatgaagggcacgagctgcttcccaaaggcccccatccaagtataggtctctacatcgtaggtgacaaagagacgctcggtgcgaggatgcgagccgatcgggaagaactggatctcccgccaccaattggaggagtggctattgatgtggtgaaagtagaagtccctgcgacgggccgaacactcgtgctggcttttgtaaaaacgtgcgcagtactggcagcggtgcacgggctgtacatcctgcacgaggttgacctgacgaccgcgcacaaggaagcagagtgggaatttgagcccctcgcctggcgggtttggctggtggtcttctacttcggctgcttgtccttgaccgtctggctgctcgaggggagttacggtggatcggaccaccacgccgcgcgagcccaaagtccagatgtccgcgcgcggcggtcggagcttgatgacaacatcgcgcagatgggagctgtccatggtctggagctcccgcggcgtcaggtcaggcgggagctcctgcaggtttacctcgcatagacgggtcagggcgcgggctagatccaggtgatacctaatttccaggggctggttggtggcggcgtcgatggcttgcaagaggccgcatccccgcggcgcgactacggtaccgcgcggcgggcggtgggccgcgggggtgtccttggatgatgcatctaaaagcggtgacgcgggcgagcccccggaggtagggggggctccggacccgccgggagagggggcaggggcacgtcggcgccgcgcgcgggcaggagctggtgctgcgcgcgtaggttgctggcgaacgcgacgacgcggcggttgatctcctgaatctggcgcctctgcgtgaagacgacgggcccggtgagcttgagcctgaaagagagttcgacagaatcaatttcggtgtcgttgacggcggcctggcgcaaaatctcctgcacgtctcctgagttgtcttgataggcgatctcggccatgaactgctcgatctcttcctcctggagatctccgcgtccggctcgctccacggtggcggcgaggtcgttggaaatgcgggccatgagctgcgagaaggcgttgaggcctccctcgttccagacgcggctgtagaccacgcccccttcggcatcgcgggcgcgcatgaccacctgcgcgagattgagctccacgtgccgggcgaagacggcgtagtttcgcaggcgctgaaagaggtagttgagggtggtggcggtgtgttctgccacgaagaagtacataacccagcgtcgcaacgtggattcgttgatatcccccaaggcctcaaggcgctccatggcctcgtagaagtccacggcgaagttgaaaaactgggagttgcgcgccgacacggttaactcctcctccagaagacggatgagctcggcgacagtgtcgcgcacctcgcgctcaaaggctacaggggcctcttcttcttcttcaatctcctcttccataagggcctccccttcttcttcttctggcggcggtgggggaggggggacacggcggcgacgacggcgcaccgggaggcggtcgacaaagcgctcgatcatctccccgcggcgacggcgcatggtctcggtgacggcgcggccgttctcgcgggggcgcagttggaagacgccgcccgtcatgtcccggttatgggttggcggggggctgccatgcggcagggatacggcgctaacgatgcatctcaacaattgttgtgtaggtactccgccgccgagggacctgagcgagtccgcatcgaccggatcggaaaacctctcgagaaaggcgtctaaccagtcacagtcgcaaggtaggctgagcaccgtggcgggcggcagcgggcggcggtcggggttgtttctggcggaggtgctgctgatgatgtaattaaagtaggcggtcttgagacggcggatggtcgacagaagcaccatgtccttgggtccggcctgctgaatgcgcaggcggtcggccatgccccaggcttcgttttgacatcggcgcaggtctttgtagtagtcttgcatgagcctttctaccggcacttcttcttctccttcctcttgtcctgcatctcttgcatctatcgctgcggcggcggcggagtttggccgtaggtggcgccctcttcctcccatgcgtgtgaccccgaagcccctcatcggctgaagcagggctaggtcggcgacaacgcgctcggctaatatggcctgctgcacctgcgtgagggtagactggaagtcatccatgtccacaaagcggtggtatgcgcccgtgttgatggtgtaagtgcagttggccataacggaccagttaacggtctggtgacccggctgcgagagctcggtgtacctgagacgcgagtaagccctcgagtcaaatacgtagtcgttgcaagtccgcaccaggtactggtatcccaccaaaaagtgcggcggcggctggcggtagaggggccagcgtagggtggccggggctccgggggcgagatcttccaacataaggcgatgatatccgtagatgtacctggacatccaggtgatgccggcggcggtggtggaggcgcgcggaaagtcgcggacgcggttccagatgttgcgcagcggcaaaaagtgctccatggtcgggacgctctggccggtcaggcgcgcgcaatcgttgacgctctagcgtgcaaaaggagagcctgtaagcgggcactcttccgtggtctggtggataaattcgcaagggtatcatggcggacgaccggggttcgagccccgtatccggccgtccgccgtgatccatgcggttaccgcccgcgtgtcgaacccaggtgtgcgacgtcagacaacgggggagtgctccttttggcttccttccaggcgcggcggctgctgcgctagcttttttggccactggccgcgcgcagcgtaagcggttaggctggaaagcgaaagcattaagtggctcgctccctgtagccggagggttattttccaagggttgagtcgcgggacccccggttcgagtctcggaccggccggactgcggcgaacgggggtttgcctccccgtcatgcaagaccccgcttgcaaattcctccggaaacagggacgagccccttttttgcttttcccagatgcatccggtgctgcggcagatgcgcccccctcctcagcagcggcaagagcaagagcagcggcagacatgcagggcaccctcccctcctcctaccgcgtcaggaggggcgacatccgcggttgacgcggcagcagatggtgattacgaacccccgcggcgccgggcccggcactacctggacttggaggagggcgagggcctggcgcggctaggagcgccctctcctgagcggcacccaagggtgcagctgaagcgtgatacgcgtgaggcgtacgtgccgcggcagaacctgtttcgcgaccgcgagggagaggagcccgaggagatgcgggatcgaaagttccacgcagggcgcgagctgcggcatggcctgaatcgcgagcggttgctgcgcgaggaggactttgagcccgacgcgcgaaccgggattagtcccgcgcgcgcacacgtggcggccgccgacctggtaaccgcatacgagcagacggtgaaccaggagattaactttcaaaaaagctttaacaaccacgtgcgtacgcttgtggcgcgcgaggaggtggctataggactgatgcatctgtgggactttgtaagcgcgctggagcaaaacccaaatagcaagccgctcatggcgcagctgttccttatagtgcagcacagcagggacaacgaggcattcagggatgcgctgctaaacatagtagagcccgagggccgctggctgctcgatttgataaacatcctgcagagcatagtggtgcaggagcgcagcttgagcctggctgacaaggtggccgccatcaactattccatgcttagcctgggcaagttttacgcccgcaagatataccataccccttacgttcccatagacaaggaggtaaagatcgaggggttctacatgcgcatggcgctgaaggtgcttaccttgagcgacgacctgggcgtttatcgcaacgagcgcatccacaaggccgtgagcgtgagccggcggcgcgagctcagcgaccgcgagctgatgcacagcctgcaaagggccctggctggcacgggcagcggcgatagagaggccgagtcctactttgacgcgggcgctgacctgcgctgggccccaagccgacgcgccctggaggcagctggggccggacctgggctggcggtggcacccgcgcgcgctggcaacgtcggcggcgtggaggaatatgacgaggacgatgagtacgagccagaggacggcgagtactaagcggtgatgtttctgatcagatgatgcaagacgcaacggacccggcggtgcgggcggcgctgcagagccagccgtccggccttaactccacggacgactggcgccaggtcatggaccgcatcatgtcgctgactgcgcgcaatcctgacgcgttccggcagcagccgcaggccaaccggctctccgcaattctggaagcggtggtcccggcgcgcgcaaaccccacgcacgagaaggtgctggcgatcgtaaacgcgctggccgaaaacagggccatccggcccgacgaggccggcctggtctacgacgcgctgcttcagcgcgtggctcgttacaacagcggcaacgtgcagaccaacctggaccggctggtgggggatgtgcgcgaggccgtggcgcagcgtgagcgcgcgcagcagcagggcaacctgggctccatggttgcactaaacgccttcctgagtacacagcccgccaacgtgccgcggggacaggaggactacaccaactttgtgagcgcactgcggctaatggtgactgagacaccgcaaagtgaggtgtaccagtctgggccagactattttttccagaccagtagacaaggcctgcagaccgtaaacctgagccaggctttcaaaaacttgcaggggctgtggggggtgcgggctcccacaggcgaccgcgcgaccgtgtctagcttgctgacgcccaactcgcgcctgttgctgctgctaatagcgcccttcacggacagtggcagcgtgtcccgggacacatacctaggtcacttgctgacactgtaccgcgaggccataggtcaggcgcatgtggacgagcatactttccaggagattacaagtgtcagccgcgcgctggggcaggaggacacgggcagcctggaggcaaccctaaactacctgctgaccaaccggcggcagaagatcccctcgttgcacagtttaaacagcgaggaggagcgcattttgcgctacgtgcagcagagcgtgagccttaacctgatgcgcgacggggtaacgcccagcgtggcgctggacatgaccgcgcgcaacatggaaccgggcatgtatgcctcaaaccggccgtttatcaaccgcctaatggactacttgcatcgcgcggccgccgtgaaccccgagtatttcaccaatgccatcttgaacccgcactggctaccgccccctggtttctacaccgggggattcgaggtgcccgagggtaacgatggattcctctgggacgacatagacgacagcgtgttttccccgcaaccgcagaccctgctagagttgcaacagcgcgagcaggcagaggcggcgctgcgaaaggaaagcttccgcaggccaagcagcttgtccgatctaggcgctgcggccccgcggtcagatgctagtagcccatttccaagcttgatagggtctcttaccagcactcgcaccacccgcccgcgcctgctgggcgaggaggagtacctaaacaactcgctgctgcagccgcagcgcgaaaaaaacctgcctccggcatttcccaacaacgggatagagagcctagtggacaagatgagtagatggaagacgtacgcgcaggagcacagggacgtgccaggcccgcgcccgcccacccgtcgtcaaaggcacgaccgtcagcggggtctggtgtgggaggacgatgactcggcagacgacagcagcgtcctggatttgggagggagtggcaacccgtttgcgcaccttcgccccaggctggggagaatgttttaaaaaaaaaaaaagcatgatgcaaaataaaaaactcaccaaggccatggcaccgagcgttggttttcttgtattccccttagtatgcggcgcgcggcgatgtatgaggaaggtcctcctccctcctacgagagtgtggtgagcgcggcgccagtggcggcggcgctgggttctcccttcgatgctcccctggacccgccgtttgtgcctccgcggtacctgcggcctaccggggggagaaacagcatccgttactctgagttggcacccctattcgacaccacccgtgtgtacctggtggacaacaagtcaacggatgtggcatccctgaactaccagaacgaccacagcaactttctgaccacggtcattcaaaacaatgactacagcccgggggaggcaagcacacagaccatcaatcttgacgaccggtcgcactggggcggcgacctgaaaaccatcctgcataccaacatgccaaatgtgaacgagttcatgtttaccaataagtttaaggcgcgggtgatggtgtcgcgcttgcctactaaggacaatcaggtggagctgaaatacgagtgggtggagttcacgctgcccgagggcaactactccgagaccatgaccatagaccttatgaacaacgcgatcgtggagcactacttgaaagtgggcagacagaacggggttctggaaagcgacatcggggtaaagtttgacacccgcaacttcagactggggtttgaccccgtcactggtcttgtcatgcctggggtatatacaaacgaagccttccatccagacatcattttgctgccaggatgcggggtggacttcacccacagccgcctgagcaacttgttgggcatccgcaagcggcaacccttccaggagggctttaggatcacctacgatgatctggagggtggtaacattcccgcactgttggatgtggacgcctaccaggcgagcttgaaagatgacaccgaacagggcgggggtggcgcaggcggcagcaacagcagtggcagcggcgcggaagagaactccaacgcggcagccgcggcaatgcagccggtggaggacatgaacgatcatgccattcgcggcgacacctttgccacacgggctgaggagaagcgcgctgaggccgaagcagcggccgaagctgccgcccccgctgcgcaacccgaggtcgagaagcctcagaagaaaccggtgatcaaacccctgacagaggacagcaagaaacgcagttacaacctaataagcaatgacagcaccttcacccagtaccgcagctggtaccttgcatacaactacggcgaccctcagaccggaatccgctcatggaccctgctttgcactcctgacgtaacctgcggctcggagcaggtctactggtcgttgccagacatgatgcaagaccccgtgaccttccgctccacgcgccagatcagcaactttccggtggtgggcgccgagctgttgcccgtgcactccaagagcttctacaacgaccaggccgtctactcccaactcatccgccagtttacctctctgacccacgtgttcaatcgctttcccgagaaccagattttggcgcgcccgccagcccccaccatcaccaccgtcagtgaaaacgttcctgctctcacagatcacgggacgctaccgctgcgcaacagcatcggaggagtccagcgagtgaccattactgacgccagacgccgcacctgcccctacgtttacaaggccctgggcatagtctcgccgcgcgtcctatcgagccgcactttttgagcaagcatgtccatccttatatcgcccagcaataacacaggctggggcctgcgcttcccaagcaagatgtttggcggggccaagaagcgctccgaccaacacccagtgcgcgtgcgcgggcactaccgcgcgccctggggcgcgcacaaacgcggccgcactgggcgcaccaccgtcgatgacgccatcgacgcggtggtggaggaggcgcgcaactacacgcccacgccgccaccagtgtccacagtggacgcggccattcagaccgtggtgcgcggagcccggcgctatgctaaaatgaagagacggcggaggcgcgtagcacgtcgccaccgccgccgacccggcactgccgcccaacgcgcggcggcggccctgcttaaccgcgcacgtcgcaccggccgacgggcggccatgcgggccgctcgaaggctggccgcgggtattgtcactgtgccccccaggtccaggcgacgagcggccgccgcagcagccgcggccattagtgctatgactcagggtcgcaggggcaacgtgtattgggtgcgcgactcggttagcggcctgcgcgtgcccgtgcgcacccgccccccgcgcaactagattgcaagaaaaaactacttagactcgtactgttgtatgtatccagcggcggcggcgcgcaacgaagctatgtccaagcgcaaaatcaaagaagagatgctccaggtcatcgcgccggagatctatggccccccgaagaaggaagagcaggattacaagccccgaaagctaaagcgggtcaaaaagaaaaagaaagatgatgatgatgaacttgacgacgaggtggaactgctgcacgctaccgcgcccaggcgacgggtacagtggaaaggtcgacgcgtaaaacgtgttttgcgacccggcaccaccgtagtctttacgcccggtgagcgctccacccgcacctacaagcgcgtgtatgatgaggtgtacggcgacgaggacctgcttgagcaggccaacgagcgcctcggggagtttgcctacggaaagcggcataaggacatgctggcgttgccgctggacgagggcaacccaacacctagcctaaagcccgtaacactgcagcaggtgctgcccgcgcttgcaccgtccgaagaaaagcgcggcctaaagcgcgagtctggtgacttggcacccaccgtgcagctgatggtacccaagcgccagcgactggaagatgtcttggaaaaaatgaccgtggaacctgggctggagcccgaggtccgcgtgcggccaatcaagcaggtggcgccgggactgggcgtgcagaccgtggacgttcagatacccactaccagtagcaccagtattgccaccgccacagagggcatggagacacaaacgtccccggttgcctcagcggtggcggatgccgcggtgcaggcggtcgctgcggccgcgtccaagacctctacggaggtgcaaacggacccgtggatgtttcgcgtttcagccccccggcgcccgcgccgttcgaggaagtacggcgccgccagcgcgctactgcccgaatatgccctacatccttccattgcgcctacccccggctatcgtggctacacctaccgccccagaagacgagcaactacccgacgccgaaccaccactggaacccgccgccgccgtcgccgtcgccagcccgtgctggccccgatttccgtgcgcagggtggctcgcgaaggaggcaggaccctggtgctgccaacagcgcgctaccaccccagcatcgtttaaaagccggtctttgtggttcttgcagatatggccctcacctgccgcctccgtttcccggtgccgggattccgaggaagaatgcaccgtaggaggggcatggccggccacggcctgacgggcggcatgcgtcgtgcgcaccaccggcggcggcgcgcgtcgcaccgtcgcatgcgcggcggtatcctgcccctccttattccactgatcgccgcggcgattggcgccgtgcccggaattgcatccgtggccttgcaggcgcagagacactgattaaaaacaagttgcatgtggaaaaatcaaaataaaaagtctggactctcacgctcgcttggtcctgtaactattttgtagaatggaagacatcaactttgcgtctctggccccgcgacacggctcgcgcccgttcatgggaaactggcaagatatcggcaccagcaatatgagcggtggcgccttcagctggggctcgctgtggagcggcattaaaaatttcggttccaccgttaagaactatggcagcaaggcctggaacagcagcacaggccagatgctgagggataagttgaaagagcaaaatttccaacaaaaggtggtagatggcctggcctctggcattagcggggtggtggacctggccaaccaggcagtgcaaaataagattaacagtaagcttgatccccgccctcccgtagaggagcctccaccggccgtggagacagtgtctccagaggggcgtggcgaaaagcgtccgcgccccgacagggaagaaactctggtgacgcaaatagacgagcctccctcgtacgaggaggcactaaagcaaggcctgcccaccacccgtcccatcgcgcccatggctaccggagtgctgggccagcacacacccgtaacgctggacctgcctccccccgccgacacccagcagaaacctgtgctgccaggcccgaccgccgttgttgtaacccgtcctagccgcgcgtccctgcgccgcgccgccagcggtccgcgatcgttgcggcccgtagccagtggcaactggcaaagcacactgaacagcatcgtgggtctgggggtgcaatccctgaagcgccgacgatgcttctgatagctaacgtgtcgtatgtgtgtcatgtatgcgtccatgtcgccgccagaggagctgctgagccgccgcgcgcccgctttccaagatggctaccccttcgatgatgccgcagtggtcttacatgcacatctcgggccaggacgcctcggagtacctgagccccgggctggtgcagtttgcccgcgccaccgagacgtacttcagcctgaataacaagtttagaaaccccacggtggcgcctacgcacgacgtgaccacagaccggtcccagcgtttgacgctgcggttcatccctgtggaccgtgaggatactgcgtactcgtacaaggcgcggttcaccctagctgtgggtgataaccgtgtgctggacatggcttccacgtactttgacatccgcggcgtgctggacaggggccctacttttaagccctactctggcactgcctacaacgccctggctcccaagggtgccccaaatccttgcgaatgggatgaagctgctactgctcttgaaataaacctagaagaagaggacgatgacaacgaagacgaagtagacgagcaagctgagcagcaaaaaactcacgtatttgggcaggcgccttattctggtataaatattacaaaggagggtattcaaataggtgtcgaaggtcaaacacctaaatatgccgataaaacatttcaacctgaacctcaaataggagaatctcagtggtacgaaacagaaattaatcatgcagctgggagagtcctaaaaaagactaccccaatgaaaccatgttacggttcatatgcaaaacccacaaatgaaaatggagggcaaggcattcttgtaaagcaacaaaatggaaagctagaaagtcaagtggaaatgcaatttttctcaactactgaggcagccgcaggcaatggtgataacttgactcctaaagtggtattgtacagtgaagatgtagatatagaaaccccagacactcatatttcttacatgcccactattaaggaaggtaactcacgagaactaatgggccaacaatctatgcccaacaggcctaattacattgcttttagggacaattttattggtctaatgtattacaacagcacgggtaatatgggtgttctggcgggccaagcatcgcagttgaatgctgttgtagatttgcaagacagaaacacagagctttcataccagcttttgcttgattccattggtgatagaaccaggtacttttctatgtggaatcaggctgttgacagctatgatccagatgttagaattattgaaaatcatggaactgaagatgaacttccaaattactgctttccactgggaggtgtgattaatacagagactcttaccaaggtaaaacctaaaacaggtcaggaaaatggatgggaaaaagatgctacagaattttcagataaaaatgaaataagagttggaaataattttgccatggaaatcaatctaaatgccaacctgtggagaaatttcctgtactccaacatagcgctgtatttgcccgacaagctaaagtacagtccttccaacgtaaaaatttctgataacccaaacacctacgactacatgaacaagcgagtggtggctcccgggctagtggactgctacattaaccttggagcacgctggtcccttgactatatggacaacgtcaacccatttaaccaccaccgcaatgctggcctgcgctaccgctcaatgttgctgggcaatggtcgctatgtgcccttccacatccaggtgcctcagaagttctttgccattaaaaacctccttctcctgccgggctcatacacctacgagtggaacttcaggaaggatgttaacatggttctgcagagctccctaggaaatgacctaagggttgacggagccagcattaagtttgatagcatttgcctttacgccaccttcttccccatggcccacaacaccgcctccacgcttgaggccatgcttagaaacgacaccaacgaccagtcctttaacgactatctctccgccgccaacatgctctaccctatacccgccaacgctaccaacgtgcccatatccatcccctcccgcaactgggcggctttccgcggctgggccttcacgcgccttaagactaaggaaaccccatcactgggctcgggctacgacccttattacacctactctggctctataccctacctagatggaaccttttacctcaaccacacctttaagaaggtggccattacctttgactcttctgtcagctggcctggcaatgaccgcctgcttacccccaacgagtttgaaattaagcgctcagttgacggggagggttacaacgttgcccagtgtaacatgaccaaagactggttcctggtacaaatgctagctaactataacattggctaccagggcttctatatcccagagagctacaaggaccgcatgtactccttctttagaaacttccagcccatgagccgtcaggtggtggatgatactaaatacaaggactaccaacaggtgggcatcctacaccaacacaacaactctggatttgttggctaccttgcccccaccatgcgcgaaggacaggcctaccctgctaacttcccctatccgcttataggcaagaccgcagttgacagcattacccagaaaaagtttctttgcgatcgcaccctttggcgcatcccattctccagtaactttatgtccatgggcgcactcacagacctgggccaaaaccttctctacgccaactccgcccacgcgctagacatgacttttgaggtggatcccatggacgagcccacccttctttatgttttgtttgaagtctttgacgtggtccgtgtgcaccagccgcaccgcggcgtcatcgaaaccgtgtacctgcgcacgcccttctcggccggcaacgccacaacataaagaagcaagcaacatcaacaacagctgccgccatgggctccagtgagcaggaactgaaagccattgtcaaagatcttggttgtgggccatattttttgggcacctatgacaagcgctttccaggctttgtttctccacacaagctcgcctgcgccatagtcaatacggccggtcgcgagactgggggcgtacactggatggcctttgcctggaacccgcactcaaaaacatgctacctctttgagccctttggcttttctgaccagcgactcaagcaggtttaccagtttgagtacgagtcactcctgcgccgtagcgccattgcttcttcccccgaccgctgtataacgctggaaaagtccacccaaagcgtacaggggcccaactcggccgcctgtggactattctgctgcatgtttctccacgcctttgccaactggccccaaactcccatggatcacaaccccaccatgaaccttattaccggggtacccaactccatgctcaacagtccccaggtacagcccaccctgcgtcgcaaccaggaacagctctacagcttcctggagcgccactcgccctacttccgcagccacagtgcgcagattaggagcgccacttctttttgtcacttgaaaaacatgtaaaaataatgtactagagacactttcaataaaggcaaatgcttttatttgtacactctcgggtgattatttacccccacccttgccgtctgcgccgtttaaaaatcaaaggggttctgccgcgcatcgctatgcgccactggcagggacacgttgcgatactggtgtttagtgctccacttaaactcaggcacaaccatccgcggcagctcggtgaagttttcactccacaggctgcgcaccatcaccaacgcgtttagcaggtcgggcgccgatatcttgaagtcgcagttggggcctccgccctgcgcgcgcgagttgcgatacacagggttgcagcactggaacactatcagcgccgggtggtgcacgctggccagcacgctcttgtcggagatcagatccgcgtccaggtcctccgcgttgctcagggcgaacggagtcaactttggtagctgccttcccaaaaagggcgcgtgcccaggctttgagttgcactcgcaccgtagtggcatcaaaaggtgaccgtgcccggtctgggcgttaggatacagcgcctgcataaaagccttgatctgcttaaaagccacctgagcctttgcgccttcagagaagaacatgccgcaagacttgccggaaaactgattggccggacaggccgcgtcgtgcacgcagcaccttgcgtcggtgttggagatctgcaccacatttcggccccaccggttcttcacgatcttggccttgctagactgctccttcagcgcgcgctgcccgttttcgctcgtcacatccatttcaatcacgtgctccttatttatcataatgcttccgtgtagacacttaagctcgccttcgatctcagcgcagcggtgcagccacaacgcgcagcccgtgggctcgtgatgcttgtaggtcacctctgcaaacgactgcaggtacgcctgcaggaatcgccccatcatcgtcacaaaggtcttgttgctggtgaaggtcagctgcaacccgcggtgctcctcgttcagccaggtcttgcatacggccgccagagcttccacttggtcaggcagtagtttgaagttcgcctttagatcgttatccacgtggtacttgtccatcagcgcgcgcgcagcctccatgcccttctcccacgcagacacgatcggcacactcagcgggttcatcaccgtaatttcactttccgcttcgctgggctcttcctcttcctcttgcgtccgcataccacgcgccactgggtcgtcttcattcagccgccgcactgtgcgcttacctcctttgccatgcttgattagcaccggtgggttgctgaaacccaccatttgtagcgccacatcttctctttcttcctcgctgtccacgattacctctggtgatggcgggcgctcgggcttgggagaagggcgcttctttttcttcttgggcgcaatggccaaatccgccgccgaggtcgatggccgcgggctgggtgtgcgcggcaccagcgcgtcttgtgatgagtcttcctcgtcctcggactcgatacgccgcctcatccgcttttttgggggcgcccggggaggcggcggcgacggggacggggacgacacgtcctccatggttgggggacgtcgcgccgcaccgcgtccgcgctcgggggtggtttcgcgctgctcctcttcccgactggccatttccttctcctataggcagaaaaagatcatggagtcagtcgagaagaaggacagcctaaccgccccctctgagttcgccaccaccgcctccaccgatgccgccaacgcgcctaccaccttccccgtcgaggcacccccgcttgaggaggaggaagtgattatcgagcaggacccaggttttgtaagcgaagacgacgaggaccgctcagtaccaacagaggataaaaagcaagaccaggacaacgcagaggcaaacgaggaacaagtcgggcggggggacgaaaggcatggcgactacctagatgtgggagacgacgtgctgttgaagcatctgcagcgccagtgcgccattatctgcgacgcgttgcaagagcgcagcgatgtgcccctcgccatagcggatgtcagccttgcctacgaacgccacctattctcaccgcgcgtaccccccaaacgccaagaaaacggcacatgcgagcccaacccgcgcctcaacttctaccccgtatttgccgtgccagaggtgcttgccacctatcacatctttttccaaaactgcaagatacccctatcctgccgtgccaaccgcagccgagcggacaagcagctggccttgcggcagggcgctgtcatacctgatatcgcctcgctcaacgaagtgccaaaaatctttgagggtcttggacgcgacgagaagcgcgcggcaaacgctctgcaacaggaaaacagcgaaaatgaaagtcactctggagtgttggtggaactcgagggtgacaacgcgcgcctagccgtactaaaacgcagcatcgaggtcacccactttgcctacccggcacttaacctaccccccaaggtcatgagcacagtcatgagtgagctgatcgtgcgccgtgcgcagcccctggagagggatgcaaatttgcaagaacaaacagaggagggcctacccgcagttggcgacgagcagctagcgcgctggcttcaaacgcgcgagcctgccgacttggaggagcgacgcaaactaatgatggccgcagtgctcgttaccgtggagcttgagtgcatgcagcggttctttgctgacccggagatgcagcgcaagctagaggaaacattgcactacacctttcgacagggctacgtacgccaggcctgcaagatctccaacgtggagctctgcaacctggtctcctaccttggaattttgcacgaaaaccgccttgggcaaaacgtgcttcattccacgctcaagggcgaggcgcgccgcgactacgtccgcgactgcgtttacttatttctatgctacacctggcagacggccatgggcgtttggcagcagtgcttggaggagtgcaacctcaaggagctgcagaaactgctaaagcaaaacttgaaggacctatggacggccttcaacgagcgctccgtggccgcgcacctggcggacatcattttccccgaacgcctgcttaaaaccctgcaacagggtctgccagacttcaccagtcaaagcatgttgcagaactttaggaactttatcctagagcgctcaggaatcttgcccgccacctgctgtgcacttcctagcgactttgtgcccattaagtaccgcgaatgccctccgccgctttggggccactgctaccttctgcagctagccaactaccttgcctaccactctgacataatggaagacgtgagcggtgacggtctactggagtgtcactgtcgctgcaacctatgcaccccgcaccgctccctggtttgcaattcgcagctgcttaacgaaagtcaaattatcggtacctttgagctgcagggtccctcgcctgacgaaaagtccgcggctccggggttgaaactcactccggggctgtggacgtcggcttaccttcgcaaatttgtacctgaggactaccacgcccacgagattaggttctacgaagaccaatcccgcccgcctaatgcggagcttaccgcctgcgtcattacccagggccacattcttggccaattgcaagccatcaacaaagcccgccaagagtttctgctacgaaagggacggggggtttacttggacccccagtccggcgaggagctcaacccaatccccccgccgccgcagccctatcagcagcagccgcgggcccttgcttcccaggatggcacccaaaaagaagctgcagctgccgccgccacccacggacgaggaggaatactgggacagtcaggcagaggaggttttggacgaggaggaggaggacatgatggaagactgggagagcctagacgaggaagcttccgaggtcgaagaggtgtcagacgaaacaccgtcaccctcggtcgcattcccctcgccggcgccccagaaatcggcaaccggttccagcatggctacaacctccgctcctcaggcgccgccggcactgcccgttcgccgacccaaccgtagatgggacaccactggaaccagggccggtaagtccaagcagccgccgccgttagcccaagagcaacaacagcgccaaggctaccgctcatggcgcgggcacaagaacgccatagttgcttgcttgcaagactgtgggggcaacatctccttcgcccgccgctttcttctctaccatcacggcgtggccttcccccgtaacatcctgcattactaccgtcatctctacagcccatactgcaccggcggcagcggcagcggcagcaacagcagcggccacacagaagcaaaggcgaccggatagcaagactctgacaaagcccaagaaatccacagcggcggcagcagcaggaggaggagcgctgcgtctggcgcccaacgaacccgtatcgacccgcgagcttagaaacaggatttttcccactctgtatgctatatttcaacagagcaggggccaagaacaagagctgaaaataaaaaacaggtctctgcgatccctcacccgcagctgcctgtatcacaaaagcgaagatcagcttcggcgcacgctggaagacgcggaggctctcttcagtaaatactgcgcgctgactcttaaggactagtttcgcgccctttctcaaatttaagcgcgaaaactacgtcatctccagcggccacacccggcgccagcacctgtcgtcagcgccattatgagcaaggaaattcccacgccctacatgtggagttaccagccacaaatgggacttgcggctggagctgcccaagactactcaacccgaataaactacatgagcgcgggaccccacatgatatcccgggtcaacggaatacgcgcccaccgaaaccgaattctcttggaacaggcggctattaccaccacacctcgtaataaccttaatccccgtagttggcccgctgccctggtgtaccaggaaagtcccgctcccaccactgtggtacttcccagagacgcccaggccgaagttcagatgactaactcaggggcgcagcttgcgggcggctttcgtcacagggtgcggtcgcccgggcagggtataactcacctgacaatcagagggcgaggtattcagctcaacgacgagtcggtgagctcctcgcttggtctccgtccggacgggacatttcagatcggcggcgccggccgctcttcattcacgcctcgtcaggcaatcctaactctgcagacctcgtcctctgagccgcgctctggaggcattggaactctgcaatttattgaggagtttgtgccatcggtctactttaaccccttctcgggacctcccggccactatccggatcaatttattcctaactttgacgcggtaaaggactcggcggacggctacgactgaatgttaagtggagaggcagagcaactgcgcctgaaacacctggtccactgtcgccgccacaagtgctttgcccgcgactccggtgagttttgctactttgaattgcccgaggatcatatcgagggcccggcgcacggcgtccggcttaccgcccagggagagcttgcccgtagcctgattcgggagtttacccagcgccccctgctagttgagcgggacaggggaccctgtgttctcactgtgatttgcaactgtcctaaccctggattacatcaagatcctctagttataactagagtacccggggatcttattccctttaactaataaaaaaaaataataaagcatcacttacttaaaatcagttagcaaatttctgtccagtttattcagcagcacctccttgccctcctcccagctctggtattgcagcttcctcctggctgcaaactttctccacaatctaaatggaatgtcagtttcctcctgttcctgtccatccgcacccactatcttcatgttgttgcagatgaagcgcgcaagaccgtctgaagataccttcaaccccgtgtatccatatgacacggaaaccggtcctccaactgtgccttttcttactcctccctttgtatcccccaatgggtttcaagagagtccccctggggtactctctttgcgcctatccgaacctctagttacctccaatggcatgcttgcgctcaaaatgggcaacggcctctctctggacgaggccggcaaccttacctcccaaaatgtaaccactgtgagcccacctctcaaaaaaaccaagtcaaacataaacctggaaatatctgcacccctcacagttacctcagaagccctaactgtggctgccgccgcacctctaatggtcgcgggcaacacactcaccatgcaatcacaggccccgctaaccgtgcacgactccaaacttagcattgccacccaaggacccctcacagtgtcagaaggaaagctagccctgcaaacatcaggccccctcaccaccaccgatagcagtacccttactatcactgcctcaccccctctaactactgccactggtagcttgggcattgacttgaaagagcccatttatacacaaaatggaaaactaggactaaagtacggggctcctttgcatgtaacagacgacctaaacactttgaccgtagcaactggtccaggtgtgactattaataatacttccttgcaaactaaagttactggagccttgggttttgattcacaaggcaatatgcaacttaatgtagcaggaggactaaggattgattctcaaaacagacgccttatacttgatgttagttatccgtttgatgctcaaaaccaactaaatctaagactaggacagggccctctttttataaactcagcccacaacttggatattaactacaacaaaggcctttacttgtttacagcttcaaacaattccaaaaagcttgaggttaacctaagcactgccaaggggttgatgtttgacgctacagccatagccattaatgcaggagatgggcttgaatttggttcacctaatgcaccaaacacaaatcccctcaaaacaaaaattggccatggcctagaatttgattcaaacaaggctatggttcctaaactaggaactggccttagttttgacagcacaggtgccattacagtaggaaacaaaaataatgataagctaactttgtggaccacaccagctccatctcctaactgtagactaaatgcagagaaagatgctaaactcactttggtcttaacaaaatgtggcagtcaaatacttgctacagtttcagttttggctgttaaaggcagtttggctccaatatctggaacagttcaaagtgctcatcttattataagatttgacgaaaatggagtgctactaaacaattccttcctggacccagaatattggaactttagaaatggagatcttactgaaggcacagcctatacaaacgctgttggatttatgcctaacctatcagcttatccaaaatctcacggtaaaactgccaaaagtaacattgtcagtcaagtttacttaaacggagacaaaactaaacctgtaacactaaccattacactaaacggtacacaggaaacaggagacacaactccaagtgcatactctatgtcattttcatgggactggtctggccacaactacattaatgaaatatttgccacatcctcttacactttttcatacattgcccaagaataaagaatcgtttgtgttatgtttcaacgtgtttatttttcaattgcagaaaatttcaagtcatttttcattcagtagtatagccccaccaccacatagcttatacagatcaccgtaccttaatcaaactcacagaaccctagtattcaacctgccacctccctcccaacacacagagtacacagtcctttctccccggctggccttaaaaagcatcatatcatgggtaacagacatattcttaggtgttatattccacacggtttcctgtcgagccaaacgctcatcagtgatattaataaactccccgggcagctcacttaagttcatgtcgctgtccagctgctgagccacaggctgctgtccaacttgcggttgcttaacgggcggcgaaggagaagtccacgcctacatgggggtagagtcataatcgtgcatcaggatagggcggtggtgctgcagcagcgcgcgaataaactgctgccgccgccgctccgtcctgcaggaatacaacatggcagtggtctcctcagcgatgattcgcaccgcccgcagcataaggcgccttgtcctccgggcacagcagcgcaccctgatctcacttaaatcagcacagtaactgcagcacagcaccacaatattgttcaaaatcccacagtgcaaggcgctgtatccaaagctcatggcggggaccacagaacccacgtggccatcataccacaagcgcaggtagattaagtggcgacccctcataaacacgctggacataaacattacctcttttggcatgttgtaattcaccacctcccggtaccatataaacctctgattaaacatggcgccatccaccaccatcctaaaccagctggccaaaacctgcccgccggctatacactgcagggaaccgggactggaacaatgacagtggagagcccaggactcgtaaccatggatcatcatgctcgtcatgatatcaatgttggcacaacacaggcacacgtgcatacacttcctcaagattacaagctcctcccgcgttagaaccatatcccagggaacaacccattcctgaatcagcgtaaatcccacactgcagggaagacctcgcacgtaactcacgttgtgcattgtcaaagtgttacattcgggcagcagcggatgatcctccagtatggtagcgcgggtttctgtctcaaaaggaggtagacgatccctactgtacggagtgcgccgagacaaccgagatcgtgttggtcgtagtgtcatgccaaatggaacgccggacgtagtcatatttcctgaagcaaaaccaggtgcgggcgtgacaaacagatctgcgtctccggtcctgccgcttagcgtgttccgtgtgatagttcaagtacaaccacactcttaagttggtcaaaagaatgctggcttcagttgtaatcaaaactccatcgcatctaatcgttctgaggaaatcatccacggtagcatatgcaaatcccaaccaagcaatgcaactggattgtgtttcaagcaggagaggagagggaagagacggaagaaccatgttaatttttttattccaaaagattatccaaaacctcaaaatgaagatctattaagtgaacgcgctcccctccggtggcgtggtcaaactctacagccaaagaacagataatggcatttgtaagatgttgcacaatggcttccaaaaggcaaacggccctcacgtccaagtggacgtaaaggctaaacccttcagggtgaatctcctctataaacattccagcaccttcaaccatgcccaaataattctcatctcgccaccttctcaatatatctctaagcaaatcccgaatattaagtccggccattgtaaaaatctgctccagagcgccctccaccttacagcctcaagcagcgaatcatgattgcaaaaattcaggttcctcacagacctgtataagattcaaaagcggaacattaacaaaaataccgcgatcccgtaggtcccttcgcagggccagctgaacataatcgtgcaggtctgcacggaccagcgcggccacttccccgccaggaaccatgacaaaagaacccacactgattatgacacgcatactcggagctatgctaaccagcgtagccccgatgtaagcttgttgcatgggcggcgatataaaatgcaaggtgctgctcaaaaaatcaggcaaagcctcgcgcaaaaaagaaagcacatcgtagtcatgctcatgcagataaaggcaggtaagctccggaaccaccacagaaaaagacaccatttttctctcaaacatgtctgcgggtttctgcataaacacaaaataaaataacaaaaaaacatttaaacattagaagcctgtcttacaacaggaaaaacaacccttataagcataagacggactacggccatgccggcgtgaccgtaaaaaaactggtcaccgtgattaaaaagcaccaccgacagctcctcggtcatgtccggagtcataatgtaagactcggtaaacacatcaggttgattcacatcggtcagtgctaaaaagcgaccgaaatagcccgggggaatacatacccgcaggcgtagagacaacattacagcccccataggaggtataacaaaattaataggagagaaaaacacataaacacctgaaaaaccctcctgcctaggcaaaatagcaccctcccgctccagaacaacatacagcgcttccacagcggcagccataacagtcagccttaccagtaaaaaagaaaacctattaaaaaaacaccactcgacacggcaccagctcaatcagtcacagtgtaaaaaagggccaagtgcagagcgagtatatataggactaaaaaatgacgtaacggttaaagtccacaaaaaacacccagaaaaccgcacgcgaacctacgcccagaaacgaaagccaaaaaacccacaacttcctcaaatcgtcacttccgttttcccacgttacgtcacttcccattttaagaaaactacaattcccaacacatacaagttactccgccctaaaacctacgtcacccgccccgttcccacgccccgcgccacgtcacaaactccaccccctcattatcatattggcttcaatccaaaataaggtatattattgatgatgttacatcgttaattaa

SEQ ID NO: 14 - protein, 23 aa, synthetic construct
MALLLCFVLLCGVVDFARSLSAS

SEQ ID NO: 15 - protein, 106 aa, synthetic construct
DIQLTQSPAIMSASPGEKVTMTCRASSSVSYMNWYQQKSGTSPKRWIYDTSKVASGVPYRFSGSGSGTSYSLTISSMEAEDAATYYCQQWSSNPLTFGAGTKLELK

SEQ ID NO: 16 - protein, 15 aa, synthetic construct
GGGGSGGGGSGGGGS

SEQ ID NO: 17 - protein, 119 aa, synthetic construct
DIKLQQSGAELARPGASVKMSCKTSGYTFTRYTMHWVKQRPGQGLEWIGYINPSRGYTNYNQKFKDKATLTTDKSSSTAYMQLSSLTSEDSAVYYCARYYDDHYCLDYWGQGTTLTVSS

SEQ ID NO: 18 - protein, 21 aa, synthetic construct
EQKLISEEDLNMHTGHHHHHH

SEQ ID NO: 19 - protein, 236 aa, synthetic construct
PRGPTIKPCPPCKECHKCPAPNLEGGPSVFIFPPNIKDVLMISLTPKVTCVVVDVSEDDPDVRISWFVNNVEVHTAQTQTHREDYNSTIRVVSALPIQHQDWMSGKEFKCKVNNKDLPSPIERTISKIKGLVRAPQVYILPPPAEQLSRKDVSLTCLVVGFNPGDISVEWTSNGHTEENYKDTAPVLDSDGSYFIYSKLDIKTSKWEKTDSFSCNVRHEGLKNYYLKKTISRTPGK

SEQ ID NO: 20 - protein, 10 aa, synthetic construct
GRKKRRQRRR

SEQ ID NO: 21 - protein, 23 aa, synthetic construct
MALLLCFVLLCGVVDFARSLSAS

SEQ ID NO: 22 - protein, 106 aa, synthetic construct; identical to SEQ ID NO: 15

SEQ ID NO: 23 - protein, 15 aa, synthetic construct
GGGGSGGGGSGGGGS

SEQ ID NO: 24 - protein, 119 aa, synthetic construct; identical to SEQ ID NO: 17

SEQ ID NO: 25 - protein, 21 aa, synthetic construct
EQKLISEEDLNMHTGHHHHHH

SEQ ID NO: 26 - protein, 266 aa, synthetic construct
PRGPTIKPCPPCKECHKCPAPNLEGGPSVFIFPPNIKDVLMISLTPKVTCVVVDVSEDDPDVRISWFVNNVEVHTAQTQTHREDYNSTIRVVSALPIQHQDWMSGKEFKCKVNNKDLPSPIERTISKIKGLVRAPQVYILPPPAEQLSRKDVSLTCLVVGFNPGDISVEWTSNGHTEENYKDTAPVLDSDGSYFIYSKLDIKTSKWEKTDSFSCNVRHEGLKNYYLKKTISRTPGKGYIPEAPRDGQAYVRKDGEWVLLSTFLSPA

SEQ ID NO: 27 - protein, 10 aa, synthetic construct
GRKKRRQRRR

SEQ ID NO: 28 - protein, 6 aa, synthetic construct
GGGGSG

SEQ ID NO: 29 - protein, 23 aa, synthetic construct
MALLLCFVLLCGVVDFARSLSAS

SEQ ID NO: 30 - protein, 118 aa, synthetic construct
DIKLQQSGAELARPGASVKMSCKTSGYTFTRYTMHWVKQRPGQGLEWIGYINPSRGYTNYNQKFKDKATLTTDKSSSTAYMQLSSLTSEDSAVYYCARYYDDHYCLDYWGQGTTLTVS

SEQ ID NO: 31 - protein, 16 aa, synthetic construct
SGGGGSGGGGSGGGGS

SEQ ID NO: 32 - protein, 106 aa, synthetic construct; identical to SEQ ID NO: 15

SEQ ID NO: 33 - protein, 21 aa, synthetic construct
EQKLISEEDLNMHTGHHHHHH

SEQ ID NO: 34 - protein, 236 aa, synthetic construct; identical to SEQ ID NO: 19

SEQ ID NO: 35 - protein, 10 aa, synthetic construct
GRKKRRQRRR

SEQ ID NO: 36 - protein, 23 aa, synthetic construct
MALLLCFVLLCGVVDFARSLSAS

SEQ ID NO: 37 - protein, 119 aa, synthetic construct; identical to SEQ ID NO: 17

SEQ ID NO: 38 - protein, 15 aa, synthetic construct
GGGGSGGGGSGGGGS

SEQ ID NO: 39 - protein, 106 aa, synthetic construct; identical to SEQ ID NO: 15

SEQ ID NO: 40 - protein, 21 aa, synthetic construct
EQKLISEEDLNMHTGHHHHHH

SEQ ID NO: 41 - protein, 236 aa, synthetic construct; identical to SEQ ID NO: 19

SEQ ID NO: 42 - protein, 33 aa, synthetic construct
GYIPEAPRDGQAYVRKDGEWVLLSTFLSPAGGG

SEQ ID NO: 43 - protein, 6 aa, synthetic construct
GGGGSG

SEQ ID NO: 44 - protein, 10 aa, synthetic construct
GRKKRRQRRR

SEQ ID NO: 45 - protein, 21 aa, synthetic construct
MALLLCFVLLCGVVDFARSLS

SEQ ID NO: 46 - protein, 107 aa, synthetic construct
DIQMTQSPSSLPASLGDRVTINCQASQDISNYLNWYQQKPGKAPKLLIYYTNKLADGVPSRFSGSGSGRDSSFTISSLESEDIGSYYCQQYYNYPWTFGPGTKLEIK

SEQ ID NO: 47 - protein, 15 aa, synthetic construct
GGGGSGGGGSGGGGS

SEQ ID NO: 48 - protein, 116 aa, synthetic construct
EVQLVESGGGLVQPGKSLKLSCEASGFTFSGYGMHWVRQAPGRGLESVAYITSSSINIKYADAVKGRFTVSRDNAKNLLFLQMNILKSEDTAMYYCARFDWDKNYWGQGTMVTVSS

SEQ ID NO: 49 - protein, 21 aa, synthetic construct
EQKLISEEDLNMHTGHHHHHH

SEQ ID NO: 50 - protein, 236 aa, synthetic construct; identical to SEQ ID NO: 19

SEQ ID NO: 51 - protein, 10 aa, synthetic construct
GRKKRRQRRR

SEQ ID NO: 52 - protein, 21 aa, synthetic construct
MALLLCFVLLCGVVDFARSLS

SEQ ID NO: 53 - protein, 107 aa, synthetic construct; identical to SEQ ID NO: 46

SEQ ID NO: 54 - protein, 15 aa, synthetic construct
GGGGSGGGGSGGGGS

SEQ ID NO: 55 - protein, 116 aa, synthetic construct; identical to SEQ ID NO: 48

SEQ ID NO: 56 - protein, 21 aa, synthetic construct
EQKLISEEDLNMHTGHHHHHH

SEQ ID NO: 57 - protein, 236 aa, synthetic construct; identical to SEQ ID NO: 19

SEQ ID NO: 58 - protein, 30 aa, synthetic construct
GYIPEAPRDGQAYVRKDGEWVLLSTFLSPA

SEQ ID NO: 59 - protein, 6 aa, synthetic construct
GGGGSG

SEQ ID NO: 60 - protein, 10 aa, synthetic construct
GRKKRRQRRR

SEQ ID NO: 61 - protein, 530 aa, synthetic construct; identical to SEQ ID NO: 1

SEQ ID NO: 62 - protein, 566 aa, synthetic construct; identical to SEQ ID NO: 2

SEQ ID NO: 63 - protein, 530 aa, synthetic construct; identical to SEQ ID NO: 3

SEQ ID NO: 64 - protein, 566 aa, synthetic construct; identical to SEQ ID NO: 4

SEQ ID NO: 65 - protein, 526 aa, synthetic construct; identical to SEQ ID NO: 9

SEQ ID NO: 66 - protein, 562 aa, synthetic construct; identical to SEQ ID NO: 10

SEQ ID NO: 67 - protein, 176 aa, synthetic construct
MEAWECLEDFSAVRNLLEQSSNSTSWFWRFLWGSSQAKLVCRIKEDYKWEFEELLKSCGELFDSLNLGHQALFQEKVIKTLDFSTPGRAAAAVAFLSFIKDKWSEETHLSGGYLLDFLAMHLWRAVVRHKNRLLLLSSVRPAIIPTEEQQQQQEEARRRRQEQSPWNPRAGLDPRE

SEQ ID NO: 68 - protein, 496 aa, synthetic construct
MERRNPSERGVPAGFSGHASVESGCETQESPATVVFRPPGDNTDGGAAAAAGGSQAAAAGAEPMEPESRPGPSGMNVVQVAELYPELRRILTITEDGQGLKGVKRERGACEATEEARNLAFSLMTRHRPECITFQQIKDNCANELDLLAQKYSIEQLTTYWLQPGDDFEEAIRVYAKVALRPDCKYKISKLVNIRNCCYISGNGAEVEIDTEDRVAFRCSMINMWPGVLGMDGVVIMNVRFTGPNFSGTVFLANTNLILHGVSFYGFNNTCVEAWTDVRVRGCAFYCCWKGVVCRPKSRASIKKCLFERCTLGILSEGNSRVRHNVASDCGCFMLVKSVAVIKHNMVCGNCEDRASQMLTCSDGNCHLLKTIHVASHSRKAWPVFEHNILTRCSLHLGNRRGVFLPYQCNLSHTKILLEPESMSKVNLNGVFDMTMKIWKVLRYDETRTRCRPCECGGKHIRNQPVMLDVTEELRPDHLVLACTRAEFGSSDEDTD

SEQ ID NO: 69 - protein, 526 aa, synthetic construct; identical to SEQ ID NO: 9

SEQ ID NO: 70 - protein, 581 aa, synthetic construct
MKRARPSEDTFNPVYPYDTETGPPTVPFLTPPFVSPNGFQESPPGVLSLRLSEPLVTSNGMLALKMGNGLSLDEAGNLTSQNVTTVSPPLKKTKSNINLEISAPLTVTSEALTVAAAAPLMVAGNTLTMQSQAPLTVHDSKLSIATQGPLTVSEGKLALQTSGPLTTTDSSTLTITASPPLTTATGSLGIDLKEPIYTQNGKLGLKYGAPLHVTDDLNTLTVATGPGVTINNTSLQTKVTGALGFDSQGNMQLNVAGGLRIDSQNRRLILDVSYPFDAQNQLNLRLGQGPLFINSAHNLDINYNKGLYLFTASNNSKKLEVNLSTAKGLMFDATAIAINAGDGLEFGSPNAPNTNPLKTKIGHGLEFDSNKAMVPKLGTGLSFDSTGAITVGNKNNDKLTLWTTPAPSPNCRLNAEKDAKLTLVLTKCGSQILATVSVLAVKGSLAPISGTVQSAHLIIRFDENGVLLNNSFLDPEYWNFRNGDLTEGTAYTNAVGFMPNLSAYPKSHGKTAKSNIVSQVYLNGDKTKPVTLTITLNGTQETGDTTPSAYSMSFSWDWSGHNYINEIFATSSYTFSYIAQE

SEQ ID NO: 71 - DNA, 37243 bp, synthetic construct
  source 1..37243: mol_type = other DNA
  5'UTR 1..103: function = L-ITR
  3'UTR 37141..37243: function = R-ITR
  regulatory 380..625: note = CMVs; regulatory_class = promoter
  gene 727..1646: note = reverse complementary sequence for delta AA 4-25 variant of E1A gene
  misc_feature 837..857: note = RNAi target site
  misc_feature 886..909: note = RNAi target site
  misc_feature 1647..1764: note = heterologous target sites for RNAi inserted into the 3-UTR of E1A, equivalent to E1A-886-909, E1A-837-857, Prot IX-7467-7487
  regulatory 1813..1910: note = promoter for E1B; regulatory_class = promoter
  CDS 1911..2441: note = E1B-19k; protein_id = 72; translation = MEAWECLEDFSAVRNLLEQSSNSTSWFWRFLWGSSQAKLVCRIKEDYKWEFEELLKSCGELFDSLNLGHQALFQEKVIKTLDFSTPGRAAAAVAFLSFIKDKWSEETHLSGGYLLDFLAMHLWRAVVRHKNRLLLLSSVRPAIIPTEEQQQQQEEARRRRQEQSPWNPRAGLDPRE
  CDS 2216..3706: note = E1B-55k; protein_id = 73; translation = MERRNPSERGVPAGFSGHASVESGCETQESPATVVFRPPGDNTDGGAAAAAGGSQAAAAGAEPMEPESRPGPSGMNVVQVAELYPELRRILTITEDGQGLKGVKRERGACEATEEARNLAFSLMTRHRPECITFQQIKDNCANELDLLAQKYSIEQLTTYWLQPGDDFEEAIRVYAKVALRPDCKYKISKLVNIRNCCYISGNGAEVEIDTEDRVAFRCSMINMWPGVLGMDGVVIMNVRFTGPNFSGTVFLANTNLILHGVSFYGFNNTCVEAWTDVRVRGCAFYCCWKGVVCRPKSRASIKKCLFERCTLGILSEGNSRVRHNVASDCGCFMLVKSVAVIKHNMVCGNCEDRASQMLTCSDGNCHLLKTIHVASHSRKAWPVFEHNILTRCSLHLGNRRGVFLPYQCNLSHTKILLEPESMSKVNLNGVFDMTMKIWKVLRYDETRTRCRPCECGGKHIRNQPVMLDVTEELRPDHLVLACTRAEFGSSDEDTD
  regulatory 3737..4320: note = IRES; regulatory_class = ribosome_binding_site
  CDS 4339..6027: note = fusion protein; protein_id = 74; translation = MALLLCFVLLCGVVDFARSLSDIQMTQSPSSLPASLGDRVTINCQASQDISNYLNWYQQKPGKAPKLLIYYTNKLADGVPSRFSGSGSGRDSSFTISSLESEDIGSYYCQQYYNYPWTFGPGTKLEIKGGGGSGGGGSGGGGSEVQLVESGGGLVQPGKSLKLSCEASGFTFSGYGMHWVRQAPGRGLESVAYITSSSINIKYADAVKGRFTVSRDNAKNLLFLQMNILKSEDTAMYYCARFDWDKNYWGQGTMVTVSSEQKLISEEDLNMHTGHHHHHHPRGPTIKPCPPCKECHKCPAPNLEGGPSVFIFPPNIKDVLMISLTPKVTCVVVDVSEDDPDVRISWFVNNVEVHTAQTQTHREDYNSTIRVVSALPIQHQDWMSGKEFKCKVNNKDLPSPIERTISKIKGLVRAPQVYILPPPAEQLSRKDVSLTCLVVGFNPGDISVEWTSNGHTEENYKDTAPVLDSDGSYFIYSKLDIKTSKWEKTDSFSCNVRHEGLKNYYLKKTISRTPGKGYIPEAPRDGQAYVRKDGEWVLLSTFLSPAGGGGSGGRKKRRQRRR
  regulatory 6094..6452: note = prMinRGC; regulatory_class = promoter
  misc_feature 6481..6543: note = inhibitory shRNA for E1A (1)
  misc_feature 6609..6666: note = inhibitory shRNA for E1A (2)
  misc_feature 6733..6789: note = inhibitory shRNA for Prot IX
  misc_feature 6856..6912: note = inhibitory shRNA for E4orf6 (1)
  misc_feature 6978..7038: note = inhibitory shRNA for E4orf6 (2)
  misc_feature 7104..7161: note = inhibitory shRNA for TP
  misc_feature 7228..7286: note = inhibitory shRNA for AdPol
  gene 9142..18064: gene = reverse complementary for polymerase Ad-Pol, part of backbone
  gene 7554..7976: note = protein IX, part of backbone
  gene 12528..18064: note = reverse complementary for terminal protein TP, part of backbone
  CDS 18100..19815: note = Prot III, penton, part of backbone; protein_id = 79; translation = MRRAAMYEEGPPPSYESVVSAAPVAAALGSPFDAPLDPPFVPPRYLRPTGGRNSIRYSELAPLFDTTRVYLVDNKSTDVASLNYQNDHSNFLTTVIQNNDYSPGEASTQTINLDDRSHWGGDLKTILHTNMPNVNEFMFTNKFKARVMVSRLPTKDNQVELKYEWVEFTLPEGNYSETMTIDLMNNAIVEHYLKVGRQNGVLESDIGVKFDTRNFRLGFDPVTGLVMPGVYTNEAFHPDIILLPGCGVDFTHSRLSNLLGIRKRQPFQEGFRITYDDLEGGNIPALLDVDAYQASLKDDTEQGGGGAGGSNSSGSGAEENSNAAAAAMQPVEDMNDHAIRGDTFATRAEEKRAEAEAAAEAAAPAAQPEVEKPQKKPVIKPLTEDSKKRSYNLISNDSTFTQYRSWYLAYNYGDPQTGIRSWTLLCTPDVTCGSEQVYWSLPDMMQDPVTFRSTRQISNFPVVGAELLPVHSKSFYNDQAVYSQLIRQFTSLTHVFNRFPENQILARPPAPTITTVSENVPALTDHGTLPLRNSIGGVQRVTITDARRRTCPYVYKALGIVSPRVLSSRTF
  CDS 22785..25643: note = hexon, part of backbone; protein_id = 80; translation = MATPSMMPQWSYMHISGQDASEYLSPGLVQFARATETYFSLNNKFRNPTVAPTHDVTTDRSQRLTLRFIPVDREDTAYSYKARFTLAVGDNRVLDMASTYFDIRGVLDRGPTFKPYSGTAYNALAPKGAPNPCEWDEAATALEINLEEEDDDNEDEVDEQAEQQKTHVFGQAPYSGINITKEGIQIGVEGQTPKYADKTFQPEPQIGESQWYETEINHAAGRVLKKTTPMKPCYGSYAKPTNENGGQGILVKQQNGKLESQVEMQFFSTTEAAAGNGDNLTPKVVLYSEDVDIETPDTHISYMPTIKEGNSRELMGQQSMPNRPNYIAFRDNFIGLMYYNSTGNMGVLAGQASQLNAVVDLQDRNTELSYQLLLDSIGDRTRYFSMWNQAVDSYDPDVRIIENHGTEDELPNYCFPLGGVINTETLTKVKPKTGQENGWEKDATEFSDKNEIRVGNNFAMEINLNANLWRNFLYSNIALYLPDKLKYSPSNVKISDNPNTYDYMNKRVVAPGLVDCYINLGARWSLDYMDNVNPFNHHRNAGLRYRSMLLGNGRYVPFHIQVPQKFFAIKNLLLLPGSYTYEWNFRKDVNMVLQSSLGNDLRVDGASIKFDSICLYATFFPMAHNTASTLEAMLRNDTNDQSFNDYLSAANMLYPIPANATNVPISIPSRNWAAFRGWAFTRLKTKETPSLGSGYDPYYTYSGSIPYLDGTFYLNHTFKKVAITFDSSVSWPGNDRLLTPNEFEIKRSVDGEGYNVAQCNMTKDWFLVQMLANYNIGYQGFYIPESYKDRMYSFFRNFQPMSRQVVDDTKYKDYQQVGILHQHNNSGFVGYLAPTMREGQAYPANFPYPLIGKTAVDSITQKKFLCDRTLWRIPFSSNFMSMGALTDLGQNLLYANSAHALDMTFEVDPMDEPTLLYVLFEVFDVVRVHQPHRGVIETVYLRTPFSAGNATT
  gene 26388..27977: note = reverse complementary for DNA-binding protein dbp, part of backbone
  CDS 28004..30427: note = 100k, part of backbone; protein_id = 75; translation = MESVEKKDSLTAPSEFATTASTDAANAPTTFPVEAPPLEEEEVIIEQDPGFVSEDDEDRSVPTEDKKQDQDNAEANEEQVGRGDERHGDYLDVGDDVLLKHLQRQCAIICDALQERSDVPLAIADVSLAYERHLFSPRVPPKRQENGTCEPNPRLNFYPVFAVPEVLATYHIFFQNCKIPLSCRANRSRADKQLALRQGAVIPDIASLNEVPKIFEGLGRDEKRAANALQQENSENESHSGVLVELEGDNARLAVLKRSIEVTHFAYPALNLPPKVMSTVMSELIVRRAQPLERDANLQEQTEEGLPAVGDEQLARWLQTREPADLEERRKLMMAAVLVTVELECMQRFFADPEMQRKLEETLHYTFRQGYVRQACKISNVELCNLVSYLGILHENRLGQNVLHSTLKGEARRDYVRDCVYLFLCYTWQTAMGVWQQCLEECNLKELQKLLKQNLKDLWTAFNERSVAAHLADIIFPERLLKTLQQGLPDFTSQSMLQNFRNFILERSGILPATCCALPSDFVPIKYRECPPPLWGHCYLLQLANYLAYHSDIMEDVSGDGLLECHCRCNLCTPHRSLVCNSQLLNESQIIGTFELQGPSPDEKSAAPGLKLTPGLWTSAYLRKFVPEDYHAHEIRFYEDQSRPPNAELTACVITQGHILGQLQAINKARQEFLLRKGRGVYLDPQSGEELNPIPPPPQPYQQQPRALASQDGTQKEAAAAAATHGRGGILGQSGRGGFGRGGGGHDGRLGEPRRGSFRGRRGVRRNTVTLGRIPLAGAPEIGNRFQHGYNLRSSGAAGTARSPTQP
  misc_feature 31811: note = delta E3, equivalent to deletion of 28137-30818 of the wild-type virus
  CDS 32330..34075: note = fiber, part of backbone; protein_id = 76; translation = MKRARPSEDTFNPVYPYDTETGPPTVPFLTPPFVSPNGFQESPPGVLSLRLSEPLVTSNGMLALKMGNGLSLDEAGNLTSQNVTTVSPPLKKTKSNINLEISAPLTVTSEALTVAAAAPLMVAGNTLTMQSQAPLTVHDSKLSIATQGPLTVSEGKLALQTSGPLTTTDSSTLTITASPPLTTATGSLGIDLKEPIYTQNGKLGLKYGAPLHVTDDLNTLTVATGPGVTINNTSLQTKVTGALGFDSQGNMQLNVAGGLRIDSQNRRLILDVSYPFDAQNQLNLRLGQGPLFINSAHNLDINYNKGLYLFTASNNSKKLEVNLSTAKGLMFDATAIAINAGDGLEFGSPNAPNTNPLKTKIGHGLEFDSNKAMVPKLGTGLSFDSTGAITVGNKNNDKLTLWTTPAPSPNCRLNAEKDAKLTLVLTKCGSQILATVSVLAVKGSLAPISGTVQSAHLIIRFDENGVLLNNSFLDPEYWNFRNGDLTEGTAYTNAVGFMPNLSAYPKSHGKTAKSNIVSQVYLNGDKTKPVTLTITLNGTQETGDTTPSAYSMSFSWDWSGHNYINEIFATSSYTFSYIAQE
  gene 34202..35365: note = reverse complementary for E4orf6/7
  gene 35286..35600: note = reverse complementary for hybrid E4orf4, Ad5/Ad11
  regulatory 35969..35971: note = reverse complementary stop codon for E4orf3; regulatory_class = terminator
  misc_feature 35969..35992: note = reverse complementary for inactivated E4orf3 locus
  gene 35989..36399: note = reverse complementary for E4orf2
  gene 36429..36815: note = reverse complementary for E4orf1
catcatcaataatataccttattttggattgaagccaatatgataatgagggggtggagtttgtgacgtggcgcggggcgtgggaacggggcgggtgacgtagtagtgtggcggaagtgtgatgttgcaagtgtggcggaacacatgtaagcgacggatgtggcaaaagtgacgtttttggtgtgcgccggtgtacacaggaagtgacaattttcgcgcggttttaggcggatgttgtagtaaatttgggcgtaaccgagtaagatttggccattttcgcgggaaaactgaataagaggaagtgaaatctgaataattttgtgttactcatagcgcgtaatctctagcatcgtaactataacggtcctaaggtagcgaaagctagtaccatggtgatgcggttttggcagtacatcaatggcggtggatagcggtccgactcacggggatttccaagtctccaccccattgacgtcaatgggagtttgttttggcaccaaaatcaacgggactttccaaaatgtcgtaacaactccgccccacggacgcaaatgggccgtaggcgtgtacggtgggcggtctatataagcccggctggtttagtgaaccgtcagatcctcgagggcgtgtagtgtatttatacccggtgagttcctcaagaggccactcttgagtgccagcgagtagagttttctcctccgagccgctccgacaccgggactgaaaatgagacatgaggtactggctgataatcttccacctcctagccattttgaaccacctacccttcacgaactgtatgatttagacgtgacggcccccgaagatcccaacgaggaggcggtttcgcagatttttcccgactctgtaatgttggcggtgcaggaagggattgacttactcacttttccgccggcgcccggttctccggagccgcctcacctttcccggcagcccgagcagccggagcagagagccttgggtccggtttctatgccaaaccttgtaccggaggtgatcgatcttacctgccacgaggctggctttccacccagtgacgacgaggatgaagagggtgaggagtttgtgttagattatgtggagcaccccgggcacggttgcaggtcttgtcattatcaccggaggaatacgggggacccagatattatgtgttcgctttgctatatgaggacctgtggcatgtttgtctacagtaagtgaaaattatgggcagtgggtgatagagtggtgggtttggtgtggtaattttttttttaatttttacagttttgtggtttaaagaattttgtattgtgatttttttaaaaggtcctgtgtctgaacctgagcctgagcccgagccagaaccggagcctgcaagacctacccgccgtcctaaaatggcgcctgctatcctgagacgcccgacatcacctgtgtctagagaatgcaatagtagtacggatagctgtgactccggtccttctaacacacctcctgagatacacccggtggtcccgctgtgccccattaaaccagttgccgtgagagttggtgggcgtcgccaggctgtggaatgtatcgaggacttgcttaacgagcctgggcaacctttggacttgagctgtaaacgccccaggccataaggtgtaaacctgtgattgcgtgtgtggttaacacacaggaggcggtttcgcagatttttacacacagaagggattgacttactcacttttacacacaggaagcattgtgagctcatatgagacccaacgcctttgtttgctgaatgagttgatgtaagtttaataaagggtgagataatgtttaacttgcatggcgtgttaaatggggcggggcttaaagggtatataatgcgccgtgggctaatcttggttacatctgacctcatggaggcttgggagtgtttggaagatttttctgctgtgcgtaacttgctggaacagagctctaacagtacctcttggttttggaggtttctgtggggctcatcccaggcaaagttagtctgcagaattaaggaggattacaagtgggaatttgaagagcttttgaaatcctgtggtgagctgtttgattctttgaatctgggtcaccaggcgcttttccaagagaaggtcatcaagactttggatttttccacaccggggcgcgctgcggctgctgttgcttttttgagttttataaaggataaatggagcgaagaaacccatctgagcggggggtacctgctggattttctggccatgcatctgtggagagcggttgtgagacacaagaatcgcctgctactgttgtcttccgtccgcccggcgataataccgacggaggagcagcagcagcagcaggaggaagccaggcggcggcggcaggagcagagcccatggaacccgagagccggcctggaccctcgggaatgaatgttgtacaggtggctgaactgtatccagaactgagacgcattttgacaattacagaggatgggcaggggctaaagggggtaaagagggagcggggggcttgtgaggctacagaggaggctaggaatctagcttttagcttaatgaccagacaccgtcctgagtgtattacttttcaacagatcaaggataattgcgctaatgagcttgatctgctggcgcagaagtattccatagagcagctgaccacttactggctgcagccaggggatgattttgaggaggctattagggtatatgcaaaggtggcacttaggccagattgcaagtacaagatcagcaaacttgtaaatatcaggaattgttgctacatttctgggaacggggccgaggtggagatagatacggaggatagggtggcctttagatgtagcatgataaatatgtggccgggggtgcttggcatggacggggtggttattatgaatgtaaggtttactggccccaattttagcggtacggttttcctggccaataccaaccttatcctacacggtgtaagcttctatgggtttaacaatacctgtgtggaagcctggaccgatgtaagggttcggggctgtgccttttactgctgctggaagggggtggtgtgtcgccccaaaagcagggcttcaattaagaaatgcctctttgaaaggtgtaccttgggtatcctgtctgagggtaactccagggtgcgccacaatgtggcctccgactgtggttgcttcatgctagtgaaaagcgtggctgtgattaagcataacatggtatgtggcaactgcgaggacagggcctctcagatgctgacctgctcggacggcaactgtcacctgctgaagaccattcacgtagccagccactctcgcaaggcctggccagtgtttgagcataacatactgacccgctgttccttgcatttgggtaacaggaggggggtgttcctaccttaccaatgcaatttgagtcacactaagatattgcttgagcccgagagcatgtccaaggtgaacctgaacggggtgtttgacatgaccatgaagatctggaaggtgctgaggtacgatgagacccgcaccaggtgcagaccctgcgagtgtggcggtaaacatattaggaaccagcctgtgatgctggatgtgaccgaggagctgaggcccgatcacttggtgctggcctgcacccgcgctgagtttggctctagcgatgaagatacagattgaggtactgaaatgtgtgggcgtggcgaattccgcccctctccctcccccccccctaacgttactggccgaagccgcttggaataaggccggtgtgcgtttgtctatatgttattttccaccatattgccgtcttttggcaatgtgagggcccggaaacctggccctgtcttcttgacgagcattcctaggggtctttcccctctcgccaaaggaatgcaaggtctgttgaatgtcgtgaaggaagcagttcctctggaagcttcttgaagacaaacaacgtctgtagcgaccctttgcaggcagcggaaccccccacctggcgacaggtgcctctgcggccaaaagccacgtgtataagatacacctgcaaaggcggcacaaccccagtgccacgttgtgagttggatagttgtggaaagagtcaaatggctctcctcaagcgtattcaacaaggggctgaaggatgcccagaaggtaccccattgtatgggatctgatctggggcctcggtgcacatgctttacatgtgtttagtcgaggttaaaaaaacgtctaggccccccgaaccacggggacgtggttttcctttgaaaaacacgatgataagcttgatcacgcgtttcgaacgatttatggccctcctgctgtgcttcgtgctcctgtgcggagtggtggatttcgccagaagtttgagtgacatccagatgacccagtctccatcatcactgcctgcctccctgggagacagagtcactatcaattgtcaggccagtcaggacattagcaattatttgaactggtaccagcagaaaccagggaaagctcctaagctcctgatctattatacaaataaattggcagatggagtcccatcaaggttcagtggcagtggctctgggagagattcttctttcactatcagcagcctggaatccgaagatattggatcttattactgtcagcagtattataactatccctggaccttcggacctggcaccaagctggaaatcaaaggaggaggagggtccggagggggcggatctggagggggaggctctgaggtgcagctggtggagtctgggggaggcttggtgcagcctggaaagtccctgaaactctcctgtgaggcctctggattcaccttcagcggctatggcatgcactgggtccgccaggctccagggagggggctggagtccgtcgcatacattactagtagtagtattaatatcaaatatgctgacgctgtgaaaggccggttcaccgtctccagagacaatgccaagaacttgctgtttctgcagatgaacattctcaagtctgaggacacagccatgtactactgtgcaagattcgactgggacaaaaattactggggccagggaaccatggtcaccgtctcctcagaacagaaactcatctcagaagaggatctgaatatgcataccggacatcatcaccatcaccatcccagagggcccacaatcaagccctgtcctccatgcaaggagtgtcacaaatgcccagctcctaacctcgagggcggaccatccgtcttcatcttccctccaaatatcaaggatgtgctcatgatctccctgacacccaaggtcacctgtgtggtggtggatgtgagcgaggatgacccagacgtccggatcagctggtttgtgaacaacgtggaagtgcacacagctcagacacagacccatagagaggattacaacagtactatccgggtggtcagtgccctccccatccagcaccaggactggatgagtggcaaggagttcaaatgcaaggtcaacaacaaagacctcccatcacccatcgagagaaccatctcaaaaattaaagggctggtcagagctccacaggtgtacatcttgcctccaccagcagagcagttgtccaggaaagatgtcagtctcacttgcctggtcgtgggcttcaaccctggagacatcagtgtggagtggaccagcaatgggcatacagaggagaactacaaggacaccgcaccagtcctggactctgacggctcttacttcatctacagcaagctcgatatcaaaacaagcaagtgggagaaaacagattccttctcatgcaacgtgagacacgagggcctgaaaaattactacctgaagaagaccatctcccggactcctggcaaaggttatattcctgaagctccaagagatgggcaagcttacgttcgtaaagatggcgaatgggtattactttctacctttttatcaccagcaggaggaggagggtccggaggcaggaagaagcggagacagcgacgaagatagaaataaaggtaccttattttcattagatttgtgtgttggttttttgtgtggcggcctcgagatgggagagcttgatgccaggcaagtccaggcaggccaggcaagtccaggcaggccaggcaagtccaggcaggccaggcaagtccaggcaggccaggcaagtccaggcaggccaggcaagtccaggcaggccaggcaagtccaggcaggccaggcaagtccaggcaggccaggcaagtccaggcaggccaggcaagtccaggcagggccaggcaagtccaggcaggccaggcaagtccaggcaggccaggcaagtccaggcaggatcgaattcgagctcgtacggtgggagggctatataagcagacctcgtttagtgaaccgtcagatcgcctggagacgaagcttgctagcggatcctcgagaaggtatattgctgttgacagtgagcgagaagggattgacttactcacttttgtgaagccacagatgaaaagtgagtaagtcaatcccttcgtgcctactgcctcggaattcactagcggatcctcgagaaggtatattgctgttgacagtgagcgaggaggcggtttcgcagattttgtgaagccacagatgaaaatctgcgaaaccgcctccgtgcctactgcctcggaattcactagcggatcctcgagaaggtatattgctgttgacagtgagcgaggaagcattgtgagctcatatgtgaagccacagatgatatgagctcacaatgcttccgtgcctactgcctcggaattcactagcggatcctcgagaaggtatattgctgttgacagtgagcgagacaggaaaccgtgtggaatagtgaagccacagatgtattccacacggtttcctgtcgtgcctactgcctcggaattcactagcggatcctcgaaaggtatattgctgttgacagtgagcgaccatgtttaatcagaggtttatagtgaagccacagatgtataaacctctgattaaacatgggtgcctactgcctcggaattcactagcggatcctcgagaaggtatattgctgttgacagtgagcgacggagtacctacacaacaattgtgaagccacagatgaattgttgtgtaggtactccggtgcctactgcctcggaattcactagcggatcctcgagaaggtatattgctgttgacagtgagcgagcgaatacgtgcagctaaacatgtgaagccacagatgatgtttagctgcacgtattcgcgtgcctactgcctcggaattcactagctagtcatatgctgcagtgtagatctaaataaagcaatagcatcacaaataaagcatttcattcactgcattctagttgtggtttgtacgcgtgatatcaattcatctatgtcgggtgcggagaaagaggtaatgaaatggcatcgactcgaagatctgggcgtggttaagggtgggaaagaatatataaggtgggggtcttatgtagttttgtatctgttttgcagcagccgccgccgccatgagcaccaactcgtttgatggaagcattgtgagctcatatttgacaacgcgcatgcccccatgggccggggtgcgtcagaatgtgatgggctccagcattgatggtcgccccgtcctgcccgcaaactctactaccttgacctacgagaccgtgtctggaacgccgttggagactgcagcctccgccgccgcttcagccgctgcagccaccgcccgcgggattgtgactgactttgctttcctgagcccgcttgcaagcagtgcagcttcccgttcatccgcccgcgatgacaagttgacggctcttttggcacaattggattctttgacccgggaacttaatgtcgtttctcagcagctgttggatctgcgccagcaggtttctgccctgaaggcttcctcccctcccaatgcggtttaaaacataaataaaaaaccagactctgtttggatttggatcaagcaagtgtcttgctgtctttatttaggggttttgcgcgcgcggtaggcccgggaccagcggtctcggtcgttgagggtcctgtgtattttttccaggacgtggtaaaggtgactctggatgttcagatacatgggcataagcccgtctctggggtggaggtagcaccactgcagagcttcatgctgcggggtggtgttgtagatgatccagtcgtagcaggagcgctgggcgtggtgcctaaaaatgtctttcagtagcaagctgattgccaggggcaggcccttggtgtaagtgtttacaaagcggttaagctgggatgggtgcatacgtggggatatgagatgcatcttggactgtatttttaggttggctatgttcccagccatatccctccggggattcatgttgtgcagaaccaccagcacagtgtatccggtgcacttgggaaatttgtcatgtagcttagaaggaaatgcgtggaagaacttggagacgcccttgtgacctccaagattttccatgcattcgtccataatgatggcaatgggcccacgggcggcggcctgggcgaagatatttctgggatcactaacgtcatagttgtgttccaggatgagatcgtcataggccatttttacaaagcgcgggcggagggtgccagactgcggtataatggttccatccggcccaggggcgtagttaccctcacagatttgcatttcccacgctttgagttcagatggggggatcatgtctacctgcggggcgatgaagaaaacggtttccggggtaggggagatcagctgggaagaaagcaggttcctgagcagctgcgacttaccgcagccggtgggcccgtaaatcacacctattaccggctgcaactggtagttaagagagctgcagctgccgtcatccctgagcaggggggccacttcgttaagcatgtccctgactcgcatgttttccctgaccaaatccgccagaaggcgctcgccgcccagcgatagcagttcttgcaaggaagcaaagtttttcaacggtttgagaccgtccgccgtaggcatgcttttgagcgtttgaccaagcagttccaggcggtcccacagctcggtcacctgctctacggcatctcgatccagcatatctcctcgtttcgcgggttggggcggctttcgctgtacggcagtagtcggtgctcgtccagacgggccagggtcatgtctttccacgggcgcagggtcctcgtcagcgtagtctgggtcacggtgaaggggtgcgctccgggctgcgcgctggccagggtgcgcttgaggctggtcctgctggtgctgaagcgctgccggtcttcgccctgcgcgtcggccaggtagcatttgaccatggtgtcatagtccagcccctccgcggcgtggcccttggcgcgcagcttgcccttggaggaggcgccgcacgaggggcagtgcagacttttgagggcgtagagcttgggcgcgagaaataccgattccggggagtaggcatccgcgccgcaggccccgcagacggtctcgcattccacgagccaggtgagctctggccgttcggggtcaaaaaccaggtttcccccatgctttttgatgcgtttcttacctctggtttccatgagccggtgtccacgctcggtgacgaaaaggctgtccgtgtccccgtatacagacttgagaggcctgtcctcgagcggtgttccgcggtcctcctcgtatagaaactcggaccactctgagacaaaggctcgcgtccaggccagcacgaaggaggctaagtgggaggggtagcggtcgttgtccactagggggtccactcgctccagggtgtgaagacacatgtcgccctcttcggcatcaaggaaggtgattggtttgtaggtgtaggccacgtgaccgggtgttcctgaaggggggctataaaagggggtgggggcgcgttcgtcctcactctcttccgcatcgctgtctgcgagggccagctgttggggtgagtactccctctgaaaagcgggcatgacttctgcgctaagattgtcagtttccaaaaacgaggaggatttgatattcacctggcccgcggtgatgcctttgagggtggccgcatccatctggtcagaaaagacaatctttttgttgtcaagcttggtggcaaacgacccgtagagggcgttggacagcaacttggcgatggagcgcagggtttggtttttgtcgcgatcggcgcgctccttggccgcgatgtttagctgcacgtattcgcgcgcaacgcaccgccattcgggaaagacggtggtgcgctcgtcgggcaccaggtgcacgcgccaaccgcggttgtgcagggtgacaaggtcaacgctggtggctacctctccgcgtaggcgctcgttggtccagcagaggcggccgcccttgcgcgagcagaatggcggtagggggtctagctgcgtctcgtccggggggtctgcgtccacggtaaagaccccgggcagcaggcgcgcgtcgaagtagtctatcttgcatccttgcaagtctagcgcctgctgccatgcgcgggcggcaagcgcgcgctcgtatgggttgagtgggggaccccatggcatggggtgggtgagcgcggaggcgtacatgccgcaaatgtcgtaaacgtagaggggctctctgagtattccaagatatgtagggtagcatcttccaccgcggatgctggcgcgcacgtaatcgtatagttcgtgcgagggagcgaggaggtcgggaccgaggttgctacgggcgggctgctctgctcggaagactatctgcctgaagatggcatgtgagttggatgatatggttggacgctggaagacgttgaagctggcgtctgtgagacctaccgcgtcacgcacgaaggaggcgtaggagtcgcgcagcttgttgaccagctcggcggtgacctgcacgtctagggcgcagtagtccagggtttccttgatgatgtcatacttatcctgtcccttttttttccacagctcgcggttgaggacaaactcttcgcggtctttccagtactcttggatcggaaacccgtcggcctccgaacggtaagagcctagcatgtagaactggttgacggcctggtaggcgcagcatcccttttctacgggtagcgcgtatgcctgcgcggccttccggagcgaggtgtgggtgagcgcaaaggtgtccctgaccatgactttgaggtactggtatttgaagtcagtgtcgtcgcatccgccctgctcccagagcaaaaagtccgtgcgctttttggaacgcggatttggcagggcgaaggtgacatcgttgaagagtatctttcccgcgcgaggcataaagttgcgtgtgatgcggaagggtcccggcacctcggaacggttgttaattacctgggcggcgagcacgatctcgtcaaagccgttgatgttgtggcccacaatgtaaagttccaagaagcgcgggatgcccttgatggaaggcaattttttaagttcctcgtaggtgagctcttcaggggagctgagcccgtgctctgaaagggcccagtctgcaagatgagggttggaagcgacgaatgagctccacaggtcacgggccattagcatttgcaggtggtcgcgaaaggtcctaaactggcgacctatggccattttttctggggtgatgcagtagaaggtaagcgggtcttgttcccagcggtcccatccaaggttcgcggctaggtctcgcgcggcagtcactagaggctcatctccgccgaacttcatgaccagcatgaagggcacgagctgcttcccaaaggcccccatccaagtataggtctctacatcgtaggtgacaaagagacgctcggtgcgaggatgcgagccgatcgggaagaactggatctcccgccaccaattggaggagtggctattgatgtggtgaaagtagaagtccctgcgacgggccgaacactcgtgctggcttttgtaaaaacgtgcgcagtactggcagcggtgcacgggctgtacatcctgcacgaggttgacctgacgaccgcgcacaaggaagcagagtgggaatttgagcccctcgcctggcgggtttggctggtggtcttctacttcggctgcttgtccttgaccgtctggctgctcgaggggagttacggtggatcggaccaccacgccgcgcgagcccaaagtccagatgtccgcgcgcggcggtcggagcttgatgacaacatcgcgcagatgggagctgtccatggtctggagctcccgcggcgtcaggtcaggcgggagctcctgcaggtttacctcgcatagacgggtcagggcgcgggctagatccaggtgatacctaatttccaggggctggttggtggcggcgtcgatggcttgcaagaggccgcatccccgcggcgcgactacggtaccgcgcggcgggcggtgggccgcgggggtgtccttggatgatgcatctaaaagcggtgacgcgggcgagcccccggaggtagggggggctccggacccgccgggagagggggcaggggcacgtcggcgccgcgcgcgggcaggagctggtgctgcgcgcgtaggttgctggcgaacgcgacgacgcggcggttgatctcctgaatctggcgcctctgcgtgaagacgacgggcccggtgagcttgagcctgaaagagagttcgacagaatcaatttcggtgtcgttgacggcggcctggcgcaaaatctcctgcacgtctcctgagttgtcttgataggcgatctcggccatgaactgctcgatctcttcctcctggagatctccgcgtccggctcgctccacggtggcggcgaggtcgttggaaatgcgggccatgagctgcgagaaggcgttgaggcctccctcgttccagacgcggctgtagaccacgcccccttcggcatcgcgggcgcgcatgaccacctgcgcgagattgagctccacgtgccgggcgaagacggcgtagtttcgcaggcgctgaaagaggtagttgagggtggtggcggtgtgttctgccacgaagaagtacataacccagcgtcgcaacgtggattcgttgatatcccccaaggcctcaaggcgctccatggcctcgtagaagtccacggcgaagttgaaaaactgggagttgcgcgccgacacggttaactcctcctccagaagacggatgagctcggcgacagtgtcgcgcacctcgcgctcaaaggctacaggggcctcttcttcttcttcaatctcctcttccataagggcctccccttcttcttcttctggcggcggtgggggaggggggacacggcggcgacgacggcgcaccgggaggcggtcgacaaagcgctcgatcatctccccgcggcgacggcgcatggtctcggtgacggcgcggccgttctcgcgggggcgcagttggaagacgccgcccgtcatgtcccggttatgggttggcggggggctgccatgcggcagggatacggcgctaacgatgcatctcaacaattgttgtgtaggtactccgccgccgagggacctgagcgagtccgcatcgaccggatcggaaaacctctcgagaaaggcgtctaaccagtcacagtcgcaaggtaggctgagcaccgtggcgggcggcagcgggcggcggtcggggttgtttctggcggaggtgctgctgatgatgtaattaaagtaggcggtcttgagacggcggatggtcgacagaagcaccatgtccttgggtccggcctgctgaatgcgcaggcggtcggccatgccccaggcttcgttttgacatcggcgcaggtctttgtagtagtcttgcatgagcctttctaccggcacttcttcttctccttcctcttgtcctgcatctcttgcatctatcgctgcggcggcggcggagtttggccgtaggtggcgccctcttcctcccatgcgtgtgaccccgaagcccctcatcggctgaagcagggctaggtcggcgacaacgcgctcggctaatatggcctgctgcacctgcgtgagggtagactggaagtcatccatgtccacaaagcggtggtatgcgcccgtgttgatggtgtaagtgcagttggccataacggaccagttaacggtctggtgacccggctgcgagagctcggtgtacctgagacgcgagtaagccctcgagtcaaatacgtagtcgttgcaagtccgcaccaggtactggtatcccaccaaaaagtgcggcggcggctggcggtagaggggccagcgtagggtggccggggctccgggggcgagatcttccaacataaggcgatgatatccgtagatgtacctggacatccaggtgatgccggcggcggtggtggaggcgcgcggaaagtcgcggacgcggttccagatgttgcgcagcggcaaaaagtgctccatggtcgggacgctctggccggtcaggcgcgcgcaatcgttgacgctctagcgtgcaaaaggagagcctgtaagcgggcactcttccgtggtctggtggataaattcgcaagggtatcatggcggacgaccggggttcgagccccgtatccggccgtccgccgtgatccatgcggttaccgcccgcgtgtcgaacccaggtgtgcgacgtcagacaacgggggagtgctccttttggcttccttccaggcgcggcggctgctgcgctagcttttttggccactggccgcgcgcagcgtaagcggttaggctggaaagcgaaagcattaagtggctcgctccctgtagccggagggttattttccaagggttgagtcgcgggacccccggttcgagtctcggaccggccggactgcggcgaacgggggtttgcctccccgtcatgcaagaccccgcttgcaaattcctccggaaacagggacgagccccttttttgcttttcccagatgcatccggtgctgcggcagatgcgcccccctcctcagcagcggcaagagcaagagcagcggcagacatgcagggcaccctcccctcctcctaccgcgtcaggaggggcgacatccgcggttgacgcggcagcagatggtgattacgaacccccgcggcgccgggcccggcactacctggacttggaggagggcgagggcctggcgcggctaggagcgccctctcctgagcggcacccaagggtgcagctgaagcgtgatacgcgtgaggcgtacgtgccgcggcagaacctgtttcgcgaccgcgagggagaggagcccgaggagatgcgggatcgaaagttccacgcagggcgcgagctgcggcatggcctgaatcgcgagcggttgctgcgcgaggaggactttgagcccgacgcgcgaaccgggattagtcccgcgcgcgcacacgtggcggccgccgacctggtaaccgcatacgagcagacggtgaaccaggagattaactttcaaaaaagctttaacaaccacgtgcgtacgcttgtggcgcgcgaggaggtggctataggactgatgcatctgtgggactttgtaagcgcgctggagcaaaacccaaatagcaagccgctcatggcgcagctgttccttatagtgcagcacagcagggacaacgaggcattcagggatgcgctgctaaacatagtagagcccgagggccgctggctgctcgatttgataaacatcctgcagagcatagtggtgcaggagcgcagcttgagcctggctgacaaggtggccgccatcaactattccatgcttagcctgggcaagttttacgcccgcaagatataccataccccttacgttcccatagacaaggaggtaaagatcgaggggttctacatgcgcatggcgctgaaggtgcttaccttgagcgacgacctgggcgtttatcgcaacgagcgcatccacaaggccgtgagcgtgagccggcggcgcgagctcagcgaccgcgagctgatgcacagcctgcaaagggccctggctggcacgggcagcggcgatagagaggccgagtcctactttgacgcgggcgctgacctgcgctgggccccaagccgacgcgccctggaggcagctggggccggacctgggctggcggtggcacccgcgcgcgctggcaacgtcggcggcgtggaggaatatgacgaggacgatgagtacgagccagaggacggcgagtactaagcggtgatgtttctgatcagatgatgcaagacgcaacggacccggcggtgcgggcggcgctgcagagccagccgtccggccttaactccacggacgactggcgccaggtcatggaccgcatcatgtcgctgactgcgcgcaatcctgacgcgttccggcagcagccgcaggccaaccggctctccgcaattctggaagcggtggtcccggcgcgcgcaaaccccacgcacgagaaggtgctggcgatcgtaaacgcgctggccgaaaacagggccatccggcccgacgaggccggcctggtctacgacgcgctgcttcagcgcgtggctcgttacaacagcggcaacgtgcagaccaacctggaccggctggtgggggatgtgcgcgaggccgtggcgcagcgtgagcgcgcgcagcagcagggcaacctgggctccatggttgcactaaacgccttcctgagtacacagcccgccaacgtgccgcggggacaggaggactacaccaactttgtgagcgcactgcggctaatggtgactgagacaccgcaaagtgaggtgtaccagtctgggccagactattttttccagaccagtagacaaggcctgcagaccgtaaacctgagccaggctttcaaaaacttgcaggggctgtggggggtgcgggctcccacaggcgaccgcgcgaccgtgtctagcttgctgacgcccaactcgcgcctgttgctgctgctaatagcgcccttcacggacagtggcagcgtgtcccgggacacatacctaggtcacttgctgacactgtaccgcgaggccataggtcaggcgcatgtggacgagcatactttccaggagattacaagtgtcagccgcgcgctggggcaggaggacacgggcagcctggaggcaaccctaaactacctgctgaccaaccggcggcagaagatcccctcgttgcacagtttaaacagcgaggaggagcgcattttgcgctacgtgcagcagagcgtgagccttaacctgatgcgcgacggggtaacgcccagcgtggcgctggacatgaccgcgcgcaacatggaaccgggcatgtatgcctcaaaccggccgtttatcaaccgcctaatggactacttgcatcgcgcggccgccgtgaaccccgagtatttcaccaatgccatcttgaacccgcactggctaccgccccctggtttctacaccgggggattcgaggtgcccgagggtaacgatggattcctctgggacgacatagacgacagcgtgttttccccgcaaccgcagaccctgctagagttgcaacagcgcgagcaggcagaggcggcgctgcgaaaggaaagcttccgcaggccaagcagcttgtccgatctaggcgctgcggccccgcggtcagatgctagtagcccatttccaagcttgatagggtctcttaccagcactcgcaccacccgcccgcgcctgctgggcgaggaggagtacctaaacaactcgctgctgcagccgcagcgcgaaaaaaacctgcctccggcatttcccaacaacgggatagagagcctagtggacaagatgagtagatggaagacgtacgcgcaggagcacagggacgtgccaggcccgcgcccgcccacccgtcgtcaaaggcacgaccgtcagcggggtctggtgtgggaggacgatgactcggcagacgacagcagcgtcctggatttgggagggagtggcaacccgtttgcgcaccttcgccccaggctggggagaatgttttaaaaaaaaaaaaagcatgatgcaaaataaaaaactcaccaaggccatggcaccgagcgttggttttcttgtattccccttagtatgcggcgcgcggcgatgtatgaggaaggtcctcctccctcctacgagagtgtggtgagcgcggcgccagtggcggcggcgctgggttctcccttcgatgctcccctggacccgccgtttgtgcctccgcggtacctgcggcctaccggggggagaaacagcatccgttactctgagttggcacccctattcgacaccacccgtgtgtacctggtggacaacaagtcaacggatgtggcatccctgaactaccagaacgaccacagcaactttctgaccacggtcattcaaaacaatgactacagcccgggggaggcaagcacacagaccatcaatcttgacgaccggtcgcactggggcggcgacctgaaaaccatcctgcataccaacatgccaaatgtgaacgagttcatgtttaccaataagtttaaggcgcgggtgatggtgtcgcgcttgcctactaaggacaatcaggtggagctgaaatacgagtgggtggagttcacgctgcccgagggcaactactccgagaccatgaccatagaccttatgaacaacgcgatcgtggagcactacttgaaagtgggcagacagaacggggttctggaaagcgacatcggggtaaagtttgacacccgcaacttcagactggggtttgaccccgtcactggtcttgtcatgcctggggtatatacaaacgaagccttccatccagacatcattttgctgccaggatgcggggtggacttcacccacagccgcctgagcaacttgttgggcatccgcaagcggcaacccttccaggagggctttaggatcacctacgatgatctggagggtggtaacattcccgcactgttggatgtggacgcctaccaggcgagcttgaaagatgacaccgaacagggcgggggtggcgcaggcggcagcaacagcagtggcagcggcgcggaagagaactccaacgcggcagccgcggcaatgcagccggtggaggacatgaacgatcatgccattcgcggcgacacctttgccacacgggctgaggagaagcgcgctgaggccgaagcagcggccgaagctgccgcccccgctgcgcaacccgaggtcgagaagcctcagaagaaaccggtgatcaaacccctgacagaggacagcaagaaacgcagttacaacctaataagcaatgacagcaccttcacccagtaccgcagctggtaccttgcatacaactacggcgaccctcagaccggaatccgctcatggaccctgctttgcactcctgacgtaacctgcggctcggagcaggtctactggtcgttgccagacatgatgcaagaccccgtgaccttccgctccacgcgccagatcagcaactttccggtggtgggcgccgagctgttgcccgtgcactccaagagcttctacaacgaccaggccgtctactcccaactcatccgccagtttacctctctgacccacgtgttcaatcgctttcccgagaaccagattttggcgcgcccgccagcccccaccatcaccaccgtcagtgaaaacgttcctgctctcacagatcacgggacgctaccgctgcgcaacagcatcggaggagtccagcgagtgaccattactgacgccagacgccgcacctgcccctacgtttacaaggccctgggcatagtctcgccgcgcgtcctatcgagccgcactttttgagcaagcatgtccatccttatatcgcccagcaataacacaggctggggcctgcgcttcccaagcaagatgtttggcggggccaagaagcgctccgaccaacacccagtgcgcgtgcgcgggcactaccgcgcgccctggggcgcgcacaaacgcggccgcactgggcgcaccaccgtcgatgacgccatcgacgcggtggtggaggaggcgcgcaactacacgcccacgccgccaccagtgtccacagtggacgcggccattcagaccgtggtgcgcggagcccggcgctatgctaaaatgaagagacggcggaggcgcgtagcacgtcgccaccgccgccgacccggcactgccgcccaacgcgcggcggcggccctgcttaaccgcgcacgtcgcaccggccgacgggcggccatgcgggccgctcgaaggctggccgcgggtattgtcactgtgccccccaggtccaggcgacgagcggccgccgcagcagccgcggccattagtgctatgactcagggtcgcaggggcaacgtgtattgggtgcgcgactcggttagcggcctgcgcgtgcccgtgcgcacccgccccccgcgcaactagattgcaagaaaaaactacttagactcgtactgttgtatgtatccagcggcggcggcgcgcaacgaagctatgtccaagcgcaaaatcaaagaagagatgctccaggtcatcgcgccggagatctatggccccccgaagaaggaagagcaggattacaagccccgaaagctaaagcgggtcaaaaagaaaaagaaagatgatgatgatgaacttgacgacgaggtggaactgctgcacgctaccgcgcccaggcgacgggtacagtggaaaggtcgacgcgtaaaacgtgttttgcgacccggcaccaccgtagtctttacgcccggtgagcgctccacccgcacctacaagcgcgtgtatgatgaggtgtacggcgacgaggacctgcttgagcaggccaacgagcgcctcggggagtttgcctacggaaagcggcataaggacatgctggcgttgccgctggacgagggcaacccaacacctagcctaaagcccgtaacactgcagcaggtgctgcccgcgcttgcaccgtccgaagaaaagcgcggcctaaagcgcgagtctggtgacttggcacccaccgtgcagctgatggtacccaagcgccagcgactggaagatgtcttggaaaaaatgaccgtggaacctgggctggagcccgaggtccgcgtgcggccaatcaagcaggtggcgccgggactgggcgtgcagaccgtggacgttcagatacccactaccagtagcaccagtattgccaccgccacagagggcatggagacacaaacgtccccggttgcctcagcggtggcggatgccgcggtgcaggcggtcgctgcggccgcgtccaagacctctacggaggtgcaaacggacccgtggatgtttcgcgtttcagccccccggcgcccgcgccgttcgaggaagtacggcgccgccagcgcgctactgcccgaatatgccctacatccttccattgcgcctacccccggctatcgtggctacacctaccgccccagaagacgagcaactacccgacgccgaaccaccactggaacccgccgccgccgtcgccgtcgccagcccgtgctggccccgatttccgtgcgcagggtggctcgcgaaggaggcaggaccctggtgctgccaacagcgcgctaccaccccagcatcgtttaaaagccggtctttgtggttcttgcagatatggccctcacctgccgcctccgtttcccggtgccgggattccgaggaagaatgcaccgtaggaggggcatggccggccacggcctgacgggcggcatgcgtcgtgcgcaccaccggcggcggcgcgcgtcgcaccgtcgcatgcgcggcggtatcctgcccctccttattccactgatcgccgcggcgattggcgccgtgcccggaattgcatccgtggccttgcaggcgcagagacactgattaaaaacaagttgcatgtggaaaaatcaaaataaaaagtctggactctcacgctcgcttggtcctgtaactattttgtagaatggaagacatcaactttgcgtctctggccccgcgacacggctcgcgcccgttcatgggaaactggcaagatatcggcaccagcaatatgagcggtggcgccttcagctggggctcgctgtggagcggcattaaaaatttcggttccaccgttaagaactatggcagcaaggcctggaacagcagcacaggccagatgctgagggataagttgaaagagcaaaatttccaacaaaaggtggtagatggcctggcctctggcattagcggggtggtggacctggccaaccaggcagtgcaaaataagattaacagtaagcttgatccccgccctcccgtagaggagcctccaccggccgtggagacagtgtctccagaggggcgtggcgaaaagcgtccgcgccccgacagggaagaaactctggtgacgcaaatagacgagcctccctcgtacgaggaggcactaaagcaaggcctgcccaccacccgtcccatcgcgcccatggctaccggagtgctgggccagcacacacccgtaacgctggacctgcctccccccgccgacacccagcagaaacctgtgctgccaggcccgaccgccgttgttgtaacccgtcctagccgcgcgtccctgcgccgcgccgccagcggtccgcgatcgttgcggcccgtagccagtggcaactggcaaagcacactgaacagcatcgtgggtctgggggtgcaatccctgaagcgccgacgatgcttctgatagctaacgtgtcgtatgtgtgtcatgtatgcgtccatgtcgccgccagaggagctgctgagccgccgcgcgcccgctttccaagatggctaccccttcgatgatgccgcagtggtcttacatgcacatctcgggccaggacgcctcggagtacctgagccccgggctggtgcagtttgcccgcgccaccgagacgtacttcagcctgaataacaagtttagaaaccccacggtggcgcctacgcacgacgtgaccacagaccggtcccagcgtttgacgctgcggttcatccctgtggaccgtgaggatactgcgtactcgtacaaggcgcggttcaccctagctgtgggtgataaccgtgtgctggacatggcttccacgtactttgacatccgcggcgtgctggacaggggccctacttttaagccctactctggcactgcctacaacgccctggctcccaagggtgccccaaatccttgcgaatgggatgaagctgctactgctcttgaaataaacctagaagaagaggacgatgacaacgaagacgaagtagacgagcaagctgagcagcaaaaaactcacgtatttgggcaggcgccttattctggtataaatattacaaaggagggtattcaaataggtgtcgaaggtcaaacacctaaatatgccgataaaacatttcaacctgaacctcaaataggagaatctcagtggtacgaaacagaaattaatcatgcagctgggagagtcctaaaaaagactaccccaatgaaaccatgttacggttcatatgcaaaacccacaaatgaaaatggagggcaaggcattcttgtaaagcaacaaaatggaaagctagaaagtcaagtggaaatgcaatttttctcaactactgaggcagccgcaggcaatggtgataacttgactcctaaagtggtattgtacagtgaagatgtagatatagaaaccccagacactcatatttcttacatgcccactattaaggaaggtaactcacgagaactaatgggccaacaatctatgcccaacaggcctaattacattgcttttagggacaattttattggtctaatgtattacaacagcacgggtaatatgggtgttctggcgggccaagcatcgcagttgaatgctgttgtagatttgcaagacagaaacacagagctttcataccagcttttgcttgattccattggtgatagaaccaggtacttttctatgtggaatcaggctgttgacagctatgatccagatgttagaattattgaaaatcatggaactgaagatgaacttccaaattactgctttccactgggaggtgtgattaatacagagactcttaccaaggtaaaacctaaaacaggtcaggaaaatggatgggaaaaagatgctacagaattttcagataaaaatgaaataagagttggaaataattttgccatggaaatcaatctaaatgccaacctgtggagaaatttcctgtactccaacatagcgctgtatttgcccgacaagctaaagtacagtccttccaacgtaaaaatttctgataacccaaacacctacgactacatgaacaagcgagtggtggctcccgggctagtggactgctacattaaccttggagcacgctggtcccttgactatatggacaacgtcaacccatttaaccaccaccgcaatgctggcctgcgctaccgctcaatgttgctgggcaatggtcgctatgtgcccttccacatccaggtgcctcagaagttctttgccattaaaaacctccttctcctgccgggctcatacacctacgagtggaacttcaggaaggatgttaacatggttctgcagagctccctaggaaatgacctaagggttgacggagccagcattaagtttgatagcatttgcctttacgccaccttcttccccatggcccacaacaccgcctccacgcttgaggccatgcttagaaacgacaccaacgaccagtcctttaacgactatctctccgccgccaacatgctctaccctatacccgccaacgctaccaacgtgcccatatccatcccctcccgcaactgggcggctttccgcggctgggccttcacgcgccttaagactaaggaaaccccatcactgggctcgggctacgacccttattacacctactctggctctataccctacctagatggaaccttttacctcaaccacacctttaagaaggtggccattacctttgactcttctgtcagctggcctggcaatgaccgcctgcttacccccaacgagtttgaaattaagcgctcagttgacggggagggttacaacgttgcccagtgtaacatgaccaaagactggttcctggtacaaatgctagctaactataacattggctaccagggcttctatatcccagagagctacaaggaccgcatgtactccttctttagaaacttccagcccatgagccgtcaggtggtggatgatactaaatacaaggactaccaacaggtgggcatcctacaccaacacaacaactctggatttgttggctaccttgcccccaccatgcgcgaaggacaggcctaccctgctaacttcccctatccgcttataggcaagaccgcagttgacagcattacccagaaaaagtttctttgcgatcgcaccctttggcgcatcccattctccagtaactttatgtccatgggcgcactcacagacctgggccaaaaccttctctacgccaactccgcccacgcgctagacatgacttttgaggtggatcccatggacgagcccacccttctttatgttttgtttgaagtctttgacgtggtccgtgtgcaccagccgcaccgcggcgtcatcgaaaccgtgtacctgcgcacgcccttctcggccggcaacgccacaacataaagaagcaagcaacatcaacaacagctgccgccatgggctccagtgagcaggaactgaaagccattgtcaaagatcttggttgtgggccatattttttgggcacctatgacaagcgctttccaggctttgtttctccacacaagctcgcctgcgccatagtcaatacggccggtcgcgagactgggggcgtacactggatggcctttgcctggaacccgcactcaaaaacatgctacctctttgagccctttggcttttctgaccagcgactcaagcaggtttaccagtttgagtacgagtcactcctgcgccgtagcgccattgcttcttcccccgaccgctgtataacgctggaaaagtccacccaaagcgtacaggggcccaactcggccgcctgtggactattctgctgcatgtttctccacgcctttgccaactggccccaaactcccatggatcacaaccccaccatgaaccttattaccggggtacccaactccatgctcaacagtccccaggtacagcccaccctgcgtcgcaaccaggaacagctctacagcttcctggagcgccactcgccctacttccgcagccacagtgcgcagattaggagcgccacttctttttgtcacttgaaaaacatgtaaaaataatgtactagagacactttcaataaaggcaaatgcttttatttgtacactctcgggtgattatttacccccacccttgccgtctgcgccgtttaaaaatcaaaggggttctgccgcgcatcgctatgcgccactggcagggacacgttgcgatactggtgtttagtgctccacttaaactcaggcacaaccatccgcggcagctcggtgaagttttcactccacaggctgcgcaccatcaccaacgcgtttagcaggtcgggcgccgatatcttgaagtcgcagttggggcctccgccctgcgcgcgcgagttgcgatacacagggttgcagcactggaacactatcagcgccgggtggtgcacgctggccagcacgctcttgtcggagatcagatccgcgtccaggtcctccgcgttgctcagggcgaacggagtcaactttggtagctgccttcccaaaaagggcgcgtgcccaggctttgagttgcactcgcaccgtagtggcatcaaaaggtgaccgtgcccggtctgggcgttaggatacagcgcctgcataaaagccttgatctgcttaaaagccacctgagcctttgcgccttcagagaagaacatgccgcaagacttgccggaaaactgattggccggacaggccgcgtcgtgcacgcagcaccttgcgtcggtgttggagatctgcaccacatttcggccccaccggttcttcacgatcttggccttgctagactgctccttcagcgcgcgctgcccgttttcgctcgtcacatccatttcaatcacgtgctccttatttatcataatgcttccgtgtagacacttaagctcgccttcgatctcagcgcagcggtgcagccacaacgcgcagcccgtgggctcgtgatgcttgtaggtcacctctgcaaacgactgcaggtacgcctgcaggaatcgccccatcatcgtcacaaaggtcttgttgctggtgaaggtcagctgcaacccgcggtgctcctcgttcagccaggtcttgcatacggccgccagagcttccacttggtcaggcagtagtttgaagttcgcctttagatcgttatccacgtggtacttgtccatcagcgcgcgcgcagcctccatgcccttctcccacgcagacacgatcggcacactcagcgggttcatcaccgtaatttcactttccgcttcgctgggctcttcctcttcctcttgcgtccgcataccacgcgccactgggtcgtcttcattcagccgccgcactgtgcgcttacctcctttgccatgcttgattagcaccggtgggttgctgaaacccaccatttgtagcgccacatcttctctttcttcctcgctgtccacgattacctctggtgatggcgggcgctcgggcttgggagaagggcgcttctttttcttcttgggcgcaatggccaaatccgccgccgaggtcgatggccgcgggctgggtgtgcgcggcaccagcgcgtcttgtgatgagtcttcctcgtcctcggactcgatacgccgcctcatccgcttttttgggggcgcccggggaggcggcggcgacggggacggggacgacacgtcctccatggttgggggacgtcgcgccgcaccgcgtccgcgctcgggggtggtttcgcgctgctcctcttcccgactggccatttccttctcctataggcagaaaaagatcatggagtcagtcgagaagaaggacagcctaaccgccccctctgagttcgccaccaccgcctccaccgatgccgccaacgcgcctaccaccttccccgtcgaggcacccccgcttgaggaggaggaagtgattatcgagcaggacccaggttttgtaagcgaagacgacgaggaccgctcagtaccaacagaggataaaaagcaagaccaggacaacgcagaggcaaacgaggaacaagtcgggcggggggacgaaaggcatggcgactacctagatgtgggagacgacgtgctgttgaagcatctgcagcgccagtgcgccattatctgcgacgcgttgcaagagcgcagcgatgtgcccctcgccatagcggatgtcagccttgcctacgaacgccacctattctcaccgcgcgtaccccccaaacgccaagaaaacggcacatgcgagcccaacccgcgcctcaacttctaccccgtatttgccgtgccagaggtgcttgccacctatcacatctttttccaaaactgcaagatacccctatcctgccgtgccaaccgcagccgagcggacaagcagctggccttgcggcagggcgctgtcatacctgatatcgcctcgctcaacgaagtgccaaaaatctttgagggtcttggacgcgacgagaagcgcgcggcaaacgctctgcaacaggaaaacagcgaaaatgaaagtcactctggagtgttggtggaactcgagggtgacaacgcgcgcctagccgtactaaaacgcagcatcgaggtcacccactttgcctacccggcacttaacctaccccccaaggtcatgagcacagtcatgagtgagctgatcgtgcgccgtgcgcagcccctggagagggatgcaaatttgcaagaacaaacagaggagggcctacccgcagttggcgacgagcagctagcgcgctggcttcaaacgcgcgagcctgccgacttggaggagcgacgcaaactaatgatggccgcagtgctcgttaccgtggagcttgagtgcatgcagcggttctttgctgacccggagatgcagcgcaagctagaggaaacattgcactacacctttcgacagggctacgtacgccaggcctgcaagatctccaacgtggagctctgcaacctggtctcctaccttggaattttgcacgaaaaccgccttgggcaaaacgtgcttcattccacgctcaagggcgaggcgcgccgcgactacgtccgcgactgcgtttacttatttctatgctacacctggcagacggccatgggcgtttggcagcagtgcttggaggagtgcaacctcaaggagctgcagaaactgctaaagcaaaacttgaaggacctatggacggccttcaacgagcgctccgtggccgcgcacctggcggacatcattttccccgaacgcctgcttaaaaccctgcaacagggtctgccagacttcaccagtcaaagcatgttgcagaactttaggaactttatcctagagcgctcaggaatcttgcccgccacctgctgtgcacttcctagcgactttgtgcccattaagtaccgcgaatgccctccgccgctttggggccactgctaccttctgcagctagccaactaccttgcctaccactctgacataatggaagacgtgagcggtgacggtctactggagtgtcactgtcgctgcaacctatgcaccccgcaccgctccctggtttgcaattcgcagctgcttaacgaaagtcaaattatcggtacctttgagctgcagggtccctcgcctgacgaaaagtccgcggctccggggttgaaactcactccggggctgtggacgtcggcttaccttcgcaaatttgtacctgaggactaccacgcccacgagattaggttctacgaagaccaatcccgcccgcctaatgcggagcttaccgcctgcgtcattacccagggccacattcttggccaattgcaagccatcaacaaagcccgccaagagtttctgctacgaaagggacggggggtttacttggacccccagtccggcgaggagctcaacccaatccccccgccgccgcagccctatcagcagcagccgcgggcccttgcttcccaggatggcacccaaaaagaagctgcagctgccgccgccacccacggacgaggaggaatactgggacagtcaggcagaggaggttttggacgaggaggaggaggacatgatggaagactgggagagcctagacgaggaagcttccgaggtcgaagaggtgtcagacgaaacaccgtcaccctcggtcgcattcccctcgccggcgccccagaaatcggcaaccggttccagcatggctacaacctccgctcctcaggcgccgccggcactgcccgttcgccgacccaaccgtagatgggacaccactggaaccagggccggtaagtccaagcagccgccgccgttagcccaagagcaacaacagcgccaaggctaccgctcatggcgcgggcacaagaacgccatagttgcttgcttgcaagactgtgggggcaacatctccttcgcccgccgctttcttctctaccatcacggcgtggccttcccccgtaacatcctgcattactaccgtcatctctacagcccatactgcaccggcggcagcggcagcggcagcaacagcagcggccacacagaagcaaaggcgaccggatagcaagactctgacaaagcccaagaaatccacagcggcggcagcagcaggaggaggagcgctgcgtctggcgcccaacgaacccgtatcgacccgcgagcttagaaacaggatttttcccactctgtatgctatatttcaacagagcaggggccaagaacaagagctgaaaataaaaaacaggtctctgcgatccctcacccgcagctgcctgtatcacaaaagcgaagatcagcttcggcgcacgctggaagacgcggaggctctcttcagtaaatactgcgcgctgactcttaaggactagtttcgcgccctttctcaaatttaagcgcgaaaactacgtcatctccagcggccacacccggcgccagcacctgtcgtcagcgccattatgagcaaggaaattcccacgccctacatgtggagttaccagccacaaatgggacttgcggctggagctgcccaagactactcaacccgaataaactacatgagcgcgggaccccacatgatatcccgggtcaacggaatacgcgcccaccgaaaccgaattctcttggaacaggcggctattaccaccacacctcgtaataaccttaatccccgtagttggcccgctgccctggtgtaccaggaaagtcccgctcccaccactgtggtacttcccagagacgcccaggccgaagttcagatgactaactcaggggcgcagcttgcgggcggctttcgtcacagggtgcggtcgcccgggcagggtataactcacctgacaatcagagggcgaggtattcagctcaacgacgagtcggtgagctcctcgcttggtctccgtccggacgggacatttcagatcggcggcgccggccgctcttcattcacgcctcgtcaggcaatcctaactctgcagacctcgtcctctgagccgcgctctggaggcattggaactctgcaatttattgaggagtttgtgccatcggtctactttaaccccttctcgggacctcccggccactatccggatcaatttattcctaactttgacgcggtaaaggactcggcggacggctacgactgaatgttaagtggagaggcagagcaactgcgcctgaaacacctggtccactgtcgccgccacaagtgctttgcccgcgactccggtgagttttgctactttgaattgcccgaggatcatatcgagggcccggcgcacggcgtccggcttaccgcccagggagagcttgcccgtagcctgattcgggagtttacccagcgccccctgctagttgagcgggacaggggaccctgtgttctcactgtgatttgcaactgtcctaaccctggattacatcaagatcctctagttataactagagtacccggggatcttattccctttaactaataaaaaaaaataataaagcatcacttacttaaaatcagttagcaaatttctgtccagtttattcagcagcacctccttgccctcctcccagctctggtattgcagcttcctcctggctgcaaactttctccacaatctaaatggaatgtcagtttcctcctgttcctgtccatccgcacccactatcttcatgttgttgcagatgaagcgcgcaagaccgtctgaagataccttcaaccccgtgtatccatatgacacggaaaccggtcctccaactgtgccttttcttactcctccctttgtatcccccaatgggtttcaagagagtccccctggggtactctctttgcgcctatccgaacctctagttacctccaatggcatgcttgcgctcaaaatgggcaacggcctctctctggacgaggccggcaaccttacctcccaaaatgtaaccactgtgagcccacctctcaaaaaaaccaagtcaaacataaacctggaaatatctgcacccctcacagttacctcagaagccctaactgtggctgccgccgcacctctaatggtcgcgggcaacacactcaccatgcaatcacaggccccgctaaccgtgcacgactccaaacttagcattgccacccaaggacccctcacagtgtcagaaggaaagctagccctgcaaacatcaggccccctcaccaccaccgatagcagtacccttactatcactgcctcaccccctctaactactgccactggtagcttgggcattgacttgaaagagcccatttatacacaaaatggaaaactaggactaaagtacggggctcctttgcatgtaacagacgacctaaacactttgaccgtagcaactggtccaggtgtgactattaataatacttccttgcaaactaaagttactggagccttgggttttgattcacaaggcaatatgcaacttaatgtagcaggaggactaaggattgattctcaaaacagacgccttatacttgatgttagttatccgtttgatgctcaaaaccaactaaatctaagactaggacagggccctctttttataaactcagcccacaacttggatattaactacaacaaaggcctttacttgtttacagcttcaaacaattccaaaaagcttgaggttaacctaagcactgccaaggggttgatgtttgacgctacagccatagccattaatgcaggagatgggcttgaatttggttcacctaatgcaccaaacacaaatcccctcaaaacaaaaattggccatggcctagaatttgattcaaacaaggctatggttcctaaactaggaactggccttagttttgacagcacaggtgccattacagtaggaaacaaaaataatgataagctaactttgtggaccacaccagctccatctcctaactgtagactaaatgcagagaaagatgctaaactcactttggtcttaacaaaatgtggcagtcaaatacttgctacagtttcagttttggctgttaaaggcagtttggctccaatatctggaacagttcaaagtgctcatcttattataagatttgacgaaaatggagtgctactaaacaattccttcctggacccagaatattggaactttagaaatggagatcttactgaaggcacagcctatacaaacgctgttggatttatgcctaacctatcagcttatccaaaatctcacggtaaaactgccaaaagtaacattgtcagtcaagtttacttaaacggagacaaaactaaacctgtaacactaaccattacactaaacggtacacaggaaacaggagacacaactccaagtgcatactctatgtcattttcatgggactggtctggccacaactacattaatgaaatatttgccacatcctcttacactttttcatacattgcccaagaataaagaatcgtttgtgttatgtttcaacgtgtttatttttcaattgcagaaaatttcaagtcatttttcattcagtagtatagccccaccaccacatagcttatacagatcaccgtaccttaatcaaactcacagaaccctagtattcaacctgccacctccctcccaacacacagagtacacagtcctttctccccggctggccttaaaaagcatcatatcatgggtaacagacatattcttaggtgttatattccacacggtttcctgtcgagccaaacgctcatcagtgatattaataaactccccgggcagctcacttaagttcatgtcgctgtccagctgctgagccacaggctgctgtccaacttgcggttgcttaacgggcggcgaaggagaagtccacgcctacatgggggtagagtcataatcgtgcatcaggatagggcggtggtgctgcagcagcgcgcgaataaactgctgccgccgccgctccgtcctgcaggaatacaacatggcagtggtctcctcagcgatgattcgcaccgcccgcagcataaggcgccttgtcctccgggcacagcagcgcaccctgatctcacttaaatcagcacagtaactgcagcacagcaccacaatattgttcaaaatcccacagtgcaaggcgctgtatccaaagctcatggcggggaccacagaacccacgtggccatcataccacaagcgcaggtagattaagtggcgacccctcataaacacgctggacataaacattacctcttttggcatgttgtaattcaccacctcccggtaccatataaacctctgattaaacatggcgccatccaccaccatcctaaaccagctggccaaaacctgcccgccggctatacactgcagggaaccgggactggaacaatgacagtggagagcccaggactcgtaaccatggatcatcatgctcgtcatgatatcaatgttggcacaacacaggcacacgtgcatacacttcctcaagattacaagctcctcccgcgttagaaccatatcccagggaacaacccattcctgaatcagcgtaaatcccacactgcagggaagacctcgcacgtaactcacgttgtgcattgtcaaagtgttacattcgggcagcagcggatgatcctccagtatggtagcgcgggtttctgtctcaaaaggaggtagacgatccctactgtacggagtgcgccgagacaaccgagatcgtgttggtcgtagtgtcatgccaaatggaacgccggacgtagtcatatttcctgaagcaaaaccaggtgcgggcgtgacaaacagatctgcgtctccggtcctgccgcttagcgtgttccgtgtgatagttcaagtacaaccacactcttaagttggtcaaaagaatgctggcttcagttgtaatcaaaactccatcgcatctaatcgttctgaggaaatcatccacggtagcatatgcaaatcccaaccaagcaatgcaactggattgtgtttcaagcaggagaggagagggaagagacggaagaaccatgttaatttttttattccaaaagattatccaaaacctcaaaatgaagatctattaagtgaacgcgctcccctccggtggcgtggtcaaactctacagccaaagaacagataatggcatttgtaagatgttgcacaatggcttccaaaaggcaaacggccctcacgtccaagtggacgtaaaggctaaacccttcagggtgaatctcctctataaacattccagcaccttcaaccatgcccaaataattctcatctcgccaccttctcaatatatctctaagcaaatcccgaatattaagtccggccattgtaaaaatctgctccagagcgccctccaccttacagcctcaagcagcgaatcatgattgcaaaaattcaggttcctcacagacctgtataagattcaaaagcggaacattaacaaaaataccgcgatcccgtaggtcccttcgcagggccagctgaacataatcgtgcaggtctgcacggaccagcgcggccacttccccgccaggaaccatgacaaaagaacccacactgattatgacacgcatactcggagctatgctaaccagcgtagccccgatgtaagcttgttgcatgggcggcgatataaaatgcaaggtgctgctcaaaaaatcaggcaaagcctcgcgcaaaaaagaaagcacatcgtagtcatgctcatgcagataaaggcaggtaagctccggaaccaccacagaaaaagacaccatttttctctcaaacatgtctgcgggtttctgcataaacacaaaataaaataacaaaaaaacatttaaacattagaagcctgtcttacaacaggaaaaacaacccttataagcataagacggactacggccatgccggcgtgaccgtaaaaaaactggtcaccgtgattaaaaagcaccaccgacagctcctcggtcatgtccggagtcataatgtaagactcggtaaacacatcaggttgattcacatcggtcagtgctaaaaagcgaccgaaatagcccgggggaatacatacccgcaggcgtagagacaacattacagcccccataggaggtataacaaaattaataggagagaaaaacacataaacacctgaaaaaccctcctgcctaggcaaaatagcaccctcccgctccagaacaacatacagcgcttccacagcggcagccataacagtcagccttaccagtaaaaaagaaaacctattaaaaaaacaccactcgacacggcaccagctcaatcagtcacagtgtaaaaaagggccaagtgcagagcgagtatatataggactaaaaaatgacgtaacggttaaagtccacaaaaaacacccagaaaaccgcacgcgaacctacgcccagaaacgaaagccaaaaaacccacaacttcctcaaatcgtcacttccgttttcccacgttacgtcacttcccattttaagaaaactacaattcccaacacatacaagttactccgccctaaaacctacgtcacccgccccgttcccacgccccgcgccacgtcacaaactccaccccctcattatcatattggcttcaatccaaaataaggtatattattgatgatgttacatcgttaattaa

SEQ ID NO: 72 - protein, 176 aa, synthetic construct; identical to SEQ ID NO: 67

SEQ ID NO: 73 - protein, 496 aa, synthetic construct; identical to SEQ ID NO: 68

SEQ ID NO: 74 - protein, 562 aa, synthetic construct; identical to SEQ ID NO: 10

SEQ ID NO: 75 - protein, 807 aa, synthetic construct
MESVEKKDSLTAPSEFATTASTDAANAPTTFPVEAPPLEEEEVIIEQDPGFVSEDDEDRSVPTEDKKQDQDNAEANEEQVGRGDERHGDYLDVGDDVLLKHLQRQCAIICDALQERSDVPLAIADVSLAYERHLFSPRVPPKRQENGTCEPNPRLNFYPVFAVPEVLATYHIFFQNCKIPLSCRANRSRADKQLALRQGAVIPDIASLNEVPKIFEGLGRDEKRAANALQQENSENESHSGVLVELEGDNARLAVLKRSIEVTHFAYPALNLPPKVMSTVMSELIVRRAQPLERDANLQEQTEEGLPAVGDEQLARWLQTREPADLEERRKLMMAAVLVTVELECMQRFFADPEMQRKLEETLHYTFRQGYVRQACKISNVELCNLVSYLGILHENRLGQNVLHSTLKGEARRDYVRDCVYLFLCYTWQTAMGVWQQCLEECNLKELQKLLKQNLKDLWTAFNERSVAAHLADIIFPERLLKTLQQGLPDFTSQSMLQNFRNFILERSGILPATCCALPSDFVPIKYRECPPPLWGHCYLLQLANYLAYHSDIMEDVSGDGLLECHCRCNLCTPHRSLVCNSQLLNESQIIGTFELQGPSPDEKSAAPGLKLTPGLWTSAYLRKFVPEDYHAHEIRFYEDQSRPPNAELTACVITQGHILGQLQAINKARQEFLLRKGRGVYLDPQSGEELNPIPPPPQPYQQQPRALASQDGTQKEAAAAAATHGRGGILGQSGRGGFGRGGGGHDGRLGEPRRGSFRGRRGVRRNTVTLGRIPLAGAPEIGNRFQHGYNLRSSGAAGTARSPTQP

SEQ ID NO: 76 - protein, 581 aa, synthetic construct; identical to SEQ ID NO: 70

SEQ ID NO: 77 - protein, 571 aa, synthetic construct
MRRAAMYEEGPPPSYESVVSAAPVAAALGSPFDAPLDPPFVPPRYLRPTGGRNSIRYSELAPLFDTTRVYLVDNKSTDVASLNYQNDHSNFLTTVIQNNDYSPGEASTQTINLDDRSHWGGDLKTILHTNMPNVNEFMFTNKFKARVMVSRLPTKDNQVELKYEWVEFTLPEGNYSETMTIDLMNNAIVEHYLKVGRQNGVLESDIGVKFDTRNFRLGFDPVTGLVMPGVYTNEAFHPDIILLPGCGVDFTHSRLSNLLGIRKRQPFQEGFRITYDDLEGGNIPALLDVDAYQASLKDDTEQGGGGAGGSNSSGSGAEENSNAAAAAMQPVEDMNDHAIRGDTFATRAEEKRAEAEAAAEAAAPAAQPEVEKPQKKPVIKPLTEDSKKRSYNLISNDSTFTQYRSWYLAYNYGDPQTGIRSWTLLCTPDVTCGSEQVYWSLPDMMQDPVTFRSTRQISNFPVVGAELLPVHSKSFYNDQAVYSQLIRQFTSLTHVFNRFPENQILARPPAPTITTVSENVPALTDHGTLPLRNSIGGVQRVTITDARRRTCPYVYKALGIVSPRVLSSRTF

SEQ ID NO: 78 - protein, 952 aa, synthetic construct
MATPSMMPQWSYMHISGQDASEYLSPGLVQFARATETYFSLNNKFRNPTVAPTHDVTTDRSQRLTLRFIPVDREDTAYSYKARFTLAVGDNRVLDMASTYFDIRGVLDRGPTFKPYSGTAYNALAPKGAPNPCEWDEAATALEINLEEEDDDNEDEVDEQAEQQKTHVFGQAPYSGINITKEGIQIGVEGQTPKYADKTFQPEPQIGESQWYETEINHAAGRVLKKTTPMKPCYGSYAKPTNENGGQGILVKQQNGKLESQVEMQFFSTTEAAAGNGDNLTPKVVLYSEDVDIETPDTHISYMPTIKEGNSRELMGQQSMPNRPNYIAFRDNFIGLMYYNSTGNMGVLAGQASQLNAVVDLQDRNTELSYQLLLDSIGDRTRYFSMWNQAVDSYDPDVRIIENHGTEDELPNYCFPLGGVINTETLTKVKPKTGQENGWEKDATEFSDKNEIRVGNNFAMEINLNANLWRNFLYSNIALYLPDKLKYSPSNVKISDNPNTYDYMNKRVVAPGLVDCYINLGARWSLDYMDNVNPFNHHRNAGLRYRSMLLGNGRYVPFHIQVPQKFFAIKNLLLLPGSYTYEWNFRKDVNMVLQSSLGNDLRVDGASIKFDSICLYATFFPMAHNTASTLEAMLRNDTNDQSFNDYLSAANMLYPIPANATNVPISIPSRNWAAFRGWAFTRLKTKETPSLGSGYDPYYTYSGSIPYLDGTFYLNHTFKKVAITFDSSVSWPGNDRLLTPNEFEIKRSVDGEGYNVAQCNMTKDWFLVQMLANYNIGYQGFYIPESYKDRMYSFFRNFQPMSRQVVDDTKYKDYQQVGILHQHNNSGFVGYLAPTMREGQAYPANFPYPLIGKTAVDSITQKKFLCDRTLWRIPFSSNFMSMGALTDLGQNLLYANSAHALDMTFEVDPMDEPTLLYVLFEVFDVVRVHQPHRGVIETVYLRTPFSAGNATT

SEQ ID NO: 79 - protein, 571 aa, synthetic construct; identical to SEQ ID NO: 77

SEQ ID NO: 80 - protein, 952 aa, synthetic construct; identical to SEQ ID NO: 78